European Patent Specification EP 3 504 334 B1, published December 6, 2023. Title: Transcription Factors to Improve Resistance to Environmental Stress in Plants. Applicant: Howe, Gregg A. Campos, Marcelo Yoshida, Yuki Board of Trustees of Michigan State University. The sequence listing filed with the application follows.

SEQUENCE LISTING (128 sequences)

SEQ ID NO: 1 - protein, 623 aa, Arabidopsis thaliana
MTDYRLQPTMNLWTTDDNASMMEAFMSSSDISTLWPPASTTTTTATTETTPTPAMEIPAQAGFNQETLQQRLQALIEGTHEGWTYAIFWQPSYDFSGASVLGWGDGYYKGEEDKANPRRRSSSPPFSTPADQEYRKKVLRELNSLISGGVAPSDDAVDEEVTDTEWFFLVSMTQSFACGAGLAGKAFATGNAVWVSGSDQLSGSGCERAKQGGVFGMHTIACIPSANGVVEVGSTEPIRQSSDLINKVRILFNFDGGAGDLSGLNWNLDPDQGENDPSMWINDPIGTPGSNEPGNGAPSSSSQLFSKSIQFENGSSSTITENPNLDPTPSPVHSQTQNPKFNNTFSRELNFSTSSSTLVKPRSGEILNFGDEGKRSSGNPDPSSYSGQTQFENKRKRSMVLNEDKVLSFGDKTAGESDHSDLEASVVKEVAVEKRPKKRGRKPANGREEPLNHVEAERQRREKLNQRFYALRAVVPNVSKMDKASLLGDAIAYINELKSKVVKTESEKLQIKNQLEEVKLELAGRKASASGGDMSSSCSSIKPVGMEIEVKIIGWDAMIRVESSKRNHPAARLMSALMDLELEVNHASMSVVNDLMIQQATVKMGFRIYTQEQLRASLISKIG

SEQ ID NO: 2 - protein, 61 aa, Arabidopsis thaliana
YDFSGASVLGWGDGYYKGEEDKANPRRRSSSPPFSTPADQEYRKKVLRELNSLISGGVAPS

SEQ ID NO: 3 - protein, 592 aa, Arabidopsis thaliana
MNGTTSSINFLTSDDDASAAAMEAFIGTNHHSSLFPPPPQQPPQPQFNEDTLQQRLQALIESAGENWTYAIFWQISHDFDSSTGDNTVILGWGDGYYKGEEDKEKKKNNTNTAEQEHRKRVIRELNSLISGGIGVSDESNDEEVTDTEWFFLVSMTQSFVNGVGLPGESFLNSRVIWLSGSGALTGSGCERAGQGQIYGLKTMVCIATQNGVVELGSSEVISQSSDLMHKVNNLFNFNNGGGNNGVEASSWGFNLNPDQGENDPALWISEPTNTGIESPARVNNGNNSNSNSKSDSHQISKLEKNDISSVENQNRQSSCLVEKDLTFQGGLLKSNETLSFCGNESSKKRTSVSKGSNNDEGMLSFSTVVRSAANDSDHSDLEASVVKEAIVVEPPEKKPRKRGRKPANGREEPLNHVEAERQRREKLNQRFYSLRAVVPNVSKMDKASLLGDAISYINELKSKLQQAESDKEEIQKKLDGMSKEGNNGKGCGSRAKERKSSNQDSTASSIEMEIDVKIIGWDVMIRVQCGKKDHPGARFMEALKELDLEVNHASLSVVNDLMIQQATVKMGSQFFNHDQLKVALMTKVGENY

SEQ ID NO: 4 - protein, 55 aa, Arabidopsis thaliana
STGDNTVILGWGDGYYKGEEDKEKKKNNTNTAEQEHRKRVIRELNSLISGGIGVS

SEQ ID NO: 5 - protein, 589 aa, Arabidopsis thaliana
MSPTNVQVTDYHLNQSKTDTTNLWSTDDDASVMEAFIGGGSDHSSLFPPLPPPPLPQVNEDNLQQRLQALIEGANENWTYAVFWQSSHGFAGEDNNNNNTVLLGWGDGYYKGEEEKSRKKKSNPASAAEQEHRKRVIRELNSLISGGVGGGDEAGDEEVTDTEWFFLVSMTQSFVKGTGLPGQAFSNSDTIWLSGSNALAGSSCERARQGQIYGLQTMVCVATENGVVELGSSEIIHQSSDLVDKVDTFFNFNNGGGEFGSWAFNLNPDQGENDPGLWISEPNGVDSGLVAAPVMNNGGNDSTSNSDSQPISKLCNGSSVENPNPKVLKSCEMVNFKNGIENGQEEDSSNKKRSPVSNNEEGMLSFTSVLPCDSNHSDLEASVAKEAESNRVVVEPEKKPRKRGRKPANGREEPLNHVEAERQRREKLNQRFYSLRAVVPNVSKMDKASLLGDAISYISELKSKLQKAESDKEELQKQIDVMNKEAGNAKSSVKDRKCLNQESSVLIEMEVDVKIIGWDAMIRIQCSKRNHPGAKFMEALKELDLEVNHASLSVVNDLMIQQATVKMGNQFFTQDQLKVALTEKVGECP

SEQ ID NO: 6 - protein, 57 aa, Arabidopsis thaliana
NNNNNTVLLGWGDGYYKGEEEKSRKKKSNPASAAEQEHRKRVIRELNSLISGGVGGG

SEQ ID NO: 7 - protein, 751 aa, Oryza sativa
MWVLLSPLLTTKNPFHPIPIPTFPLLLFSSSLVGVLFQIKSNLEEEEIEIKSMNLWTDDNASMMEAFMASADLPAFPWGAASTPPPPPPPPHHHHQQQQQQVLPPPAAAPAAAAFNQDTLQQRLQSIIEGSRETWTYAIFWQSSIDVSTGASLLGWGDGYYKGCDDDKRKQRSSTPAAAAEQEHRKRVLRELNSLIAGAGAAPDEAVEEEVTDTEWFFLVSMTQSFPNGLGLPGQALFAAQPTWIATGLSSAPCDRARQAYTFGLRTMVCLPLATGVLELGSTDVIFQTGDSIPRIRALFNLSAAAASSWPPHPDAASADPSVLWLADAPPMDMKDSISAADISVSKPPPPPPHQIQHFENGSTSTLTENPSPSVHAPTPSQPAAPPQRQQQQQQSSQAQQGPFRRELNFSDFASNGGAAAPPFFKPETGEILNFGNDSSSGRRNPSPAPPAATASLTTAPGSLFSQHTPTLTAAANDAKSNNQKRSMEATSRASNTNNHPAATANEGMLSFSSAPTTRPSTGTGAPAKSESDHSDLEASVREVESSRVVAPPPEAEKRPRKRGRKPANGREEPLNHVEAERQRREKLNQRFYALRAVVPNVSKMDKASLLGDAISYINELRGKLTALETDKETLQSQMESLKKERDARPPAPSGGGGDGGARCHAVEIEAKILGLEAMIRVQCHKRNHPAARLMTALRELDLDVYHASVSVVKDLMIQQVAVKMASRVYSQDQLNAALYTRIAEPGTAAR

SEQ ID NO: 8 - protein, 52 aa, Oryza sativa
STGASLLGWGDGYYKGCDDDKRKQRSSTPAAAAEQEHRKRVLRELNSLIAGA

SEQ ID NO: 9 - protein, 705 aa, Zea mays
MNLWTDDNASMMEAFMASADLPTFPWGAPAGGGNSSAAAASPPPPQMPAATAPGFNQDTLQQRLQAMIEGSRETWTYAIFWQSSLDSATGASLLGWGDGYYKGCDEDKRKQKPLTPSAQAEQEHRKRVLRELNSLISGAAAAPDEAVEEEVTDTEWFFLVSMTQSFLNGSGLPGQALFAGQPTWIASGLSSAPCERARQAYNFGLRTMVCFPVGTGVLELGSTDVVFKTAESMAKIRSLFGGGAGGGSWPPVQPQAPSSQQPAAGADHAETDPSMLWLADAPVMDIKDSLSHPSAEISVSKPPPHPPQIHFENGSTSTLTENPSPSVHAPPPPPAPAAPQQRQHQHQNQAHQGPFRRELNFSDFASTPSLAATPPFFKPESGEILSFGADSNARRNPSPVPPAATASLTTAPGSLFSQHTATMTAAAANDAKNNNKRSMEATSRASNTNHHPAATANEGMLSFSSAPTTRPSTGTGAPAKSESDHSDLDASVREVESSRVVAPPPEAEKRPRKRGRKPANGREEPLNHVEAERQRREKLNQRFYALRAVVPNVSKMDKASLLGDAISYINELRGKLTSLETDKETLQTQVEALKKERDARPPSHSAGLGGHDGGPRCHAVEIDAKILGLEAMIRVQCHKRNHPSARLMTALRELDLDVYHASVSVVKDLMIQQVAVKMASRVYTQDQLSAALYSRLAEPGSAMGR

SEQ ID NO: 10 - protein, 52 aa, Zea mays
ATGASLLGWGDGYYKGCDEDKRKQKPLTPSAQAEQEHRKRVLRELNSLISGA

SEQ ID NO: 11 - protein, 703 aa, Zea mays
MNLWTDDNASMMEAFMASADLPAYPWGAPAGGGNPPPPQMPPAMAMAPGFNQDTLQQRLQAMIEGSRETWTYAIFWQSSLDAATGASLLGWGDGYYKGCDDDKRRHRPPLTPAAQAEQEHRKRVLRELNSLISGGASAAPAPAPDEAVEEEVTDTEWFFLVSMTQSFLNGSGLPGQALFAGHHTWIAAGLSSAPCDRARQAYNFGLRTMVCFPVGTGVLELGSTDVVFQTAETMAKIRSLFGGGPGGGSWPPVQPQAAPQQQHAAEADQAAETDPSVLWLADAPVVDIKDSYSHPSAAEISVSKPPPPPPPPQIHFENGSTSTLTENPSPSVHAPPAPPAPPQRQQQNQGPFRRELNFSDFASNPSLAAAPPFFKPESGEILSFGVDSNAQRNPSPAPPASLTTAPGSLFSQSQHTATAAANDAKNNNNNNKRSMEATSLASNTNHHPAAAANEGMLSFSSAPTARPSAGTGAPAKSESDHSDLDASVREVESSRVVAPPPEAEKRPRKRGRKPANGREEPLNHVEAERQRREKLNQRFYALRAVVPNVSKMDKASLLGDAISYINELRGKLTSLESDRETLQAQVEALKKERDARPHPHPAAGLGGHDAGGPRCHAVEIDAKILGLEAMIRVQCHKRNHPSARLMTALRELDLDVYHASVSVVKDLMIQQVAVKMASRMYSQDQLSAALYSRLAEPGSVMGR

SEQ ID NO: 12 - protein, 53 aa, Zea mays
ATGASLLGWGDGYYKGCDDDKRRHRPPLTPAAQAEQEHRKRVLRELNSLISGG

SEQ ID NO: 13 - protein, 706 aa, Brachypodium distachyon
MNLWTDDNASMMEAFMASAADLPTFPWGAAAATPPPPAAVMPQQPAFNQDTLQQRLQAIIEGSRETWTYAIFWQSSTDAGAGASLLGWGDGYYKGCDDADKRARQQPTPASAAEQEHRKRVLRELNSLIAGGGAAAPDEAVEEEVTDTEWFFLVSMTQSFPNGMGLPGQALYTRQPTWIASGLASAPCERARQAYTFGLRTMVCIPVGTGVLELGATEVIFQTADSLGRIRSLFNLNGGGGGGGAGSSWPPVAPHQQHGGDQAETDPSVLWLTDAPVGDMKESPSVEISVSKPPPPPQIHHFENGSTSTLTENAGPSLHAHQQPATLAPAAPPRQNQHPHQLQLQHQQSQQQQQQQQGPFRRELNFSDFATNASVTVTPPFFKPESGEILNFGADSTSRRNPSPAPPAAAASLTTAPGSLFSQHTATVTAPTNEAKNNPKRSMEATSRASNTNHHPSATANEGMLSFSSAPTTRPSTGTGAPAKSESDHSDLEASVREVESSRVVPPPEEKRPRKRGRKPANGREEPLNHVEAERQRREKLNQRFYALRAVVPNVSKMDKASLLGDAISYINELRGKMTALESDKDTLHSQIEALKKERDARPVAPLSGVHDSGPRCHAVEIEAKILGLEAMIRVQCHKRNHPAAKLMTALRELDLDVYHASVSVVKDIMIQQVAVKMPNRVYSQDQLNAALYSRLAEPGAPVPIR

SEQ ID NO: 14 - protein, 52 aa, Brachypodium distachyon
AGASLLGWGDGYYKGCDDADKRARQQPTPASAAEQEHRKRVLRELNSLIAGG

SEQ ID NO: 15 - protein, 707 aa, Sorghum bicolor
MNLWTDDNASMMEAFMASADLPTFPWGATAGGGNSSAAAATPPPPPQMPAAAMAPGFNQDTLQQRLQAMIEGSSETWTYAIFWQSSLDAATGASLLGWGDGYYKGCDDDKRKQRPLTPAAQAEQEHRKRVLRELNSLISGAAAAPDEAVEEEVTDTEWFFLVSMTQSFLNGSGLPGQALFAGQPTWIASGLSSAPCERARQAYNFGLRTMVCFPVGTGVLELGSTDVVFQTAESMAKIRSLFGGGAGGGSWPPPQAPSHQQPAAGPDQAETDLWLADAPVMDIKDSMSHPSAEISVSKPPPPPPPPQIHFENASTSTLTENPSPSVHAAPPQPAPAAAPQRQHQHQNQAHQGPFRRELNFSDFASTNPSSLAATPPFFKPESGEILSFGADSNARRNPSPAPPAATASLTTAPGSLFSQHTATMTQAAAANDAKNNNKRSMEATSRASNTNHHPAATANEGMLSFSSAPTTRPSTGTGAPAKSESDHSDLDASVREVESSRVVAPPPEAEKRPRKRGRKPANGREEPLNHVEAERQRREKLNQRFYALRAVVPNVSKMDKASLLGDAISYINELRGKLTSLESDKDTLQAQIEALKKERDARPPAHAAGLGGHDGGPRCHAVEIDAKILGLEAMIRVQCHKRNHPSARLMTALRELDLDVYHASVSVVKDLMIQQVAVKMASRIYSQDQLNAALYSRLAEPGSAMGR

SEQ ID NO: 16 - protein, 51 aa, Sorghum bicolor
ATGASLLGWGDGYYKGCDDDKRKQRPLTPAAQAEQEHRKRVLRELNSLISG

SEQ ID NO: 17 - protein, 462 aa, Camelina sativa
  VARIANT (1)...(462): Xaa = Any Amino Acid
MTDYRLQPTMNLWTTDDNASMMEAFISSSDISTLWPMATTTTTTTTATTSAPATAMDIPAPAGFNQETLQQRLQALIEGTNEGWTYAIFWQPSYDFSGASVLGWGDGYYKGEEDKAKPRQRSSSPPFSTPADQEYRKKVLRELNSLISGGVAPSDDAVDEEVTDTEWFFLVSMTQSFACGAGLAGRAFSTGNAVWVSGSDQLSGSGCERAKQGGVFGMQTIACIPSANGVVEVGSTEQIRQSSDLINKVRVLFNLDGGAGDLSGLDWNLDPDQGENDPSMWINDPIGAPGSNEPGNGAPSSSSQLFSKSIQFENGSSSTITENPNPDPTPSPVHSQTQNPKFSNNFSRELNFSTSSSTLVKPRSGEILSFGDDGKRGSGNPDPSSYSGQTQFENKRKKSPNEDKVLSFGDKTTGESDHSDLEASVVKEVAVEKRPKKRGRKPANGREEPLNXMIYVIHSPNP

SEQ ID NO: 18 - protein, 80 aa, Camelina sativa
QRLQALIEGTNEGWTYAIFWQPSYDFSGASVLGWGDGYYKGEEDKAKPRQRSSSPPFSTPADQEYRKKVLRELNSLISGG

SEQ ID NO: 19 - protein, 689 aa, Solanum lycopersicum
MTEYSLPTMNLWNNSTSDDNVSMMEAFMSSDLSFWATNNSTSAAVVGVNSNLPHASSNTPSVFAPSSSTSASTLSAAATVDASKSMPFFNQETLQQRLQALIDGARETWTYAIFWQSSVVDFSSPSVLGWGDGYYKGEEDKAKRKLSVSSPAYIAEQEHRKKVLRELNSLISGAPPGTDDAVDEEVTDTEWFFLISMTQSFVNGSGLPGQALYSSSPIWVAGTEKLAASHCERVRQAQGFGLQTIVCIPSANGVVELGSTELIVQSSDLMNKVRVLFNFSNDLGSGSWAVQPESDPSALWLTDPSSSGMEVRESLNTVQTNSVPSSNSNKQIAYGNENNHPSGNGQSCYNQQQQKNPPQQQTQGFFTRELNFSEFGFDGSSNRNGNSSVSCKPESGEILNFGDSTKKSASSANVNLFTGQSQFGAGEENNNKNKKRSATSRGSNEEGMLSFVSGTVLPSSGMKSGGGGGEDSEHSDLEASVVKEADSSRVVEPEKRPRKRGRKPANGREEPLNHVEAERQRREKLNQRFYALRAVVPNVSKMDKASLLGDAISYINELKSKLQNTESDKEDLKSQIEDLKKESRRPGPPPPPNQDLKMSSHTGGKIVDVDIDVKIIGWDAMIRIQCNKKNHPAARLMAALMELDLDVHHASVSVVNDLMIQQATVKMGSRHYTEEQLRVALTSKIAETH

SEQ ID NO: 20 - protein, 53 aa, Solanum lycopersicumv
FSSPSVLGWGDGYYKGEEDKAKRKLSVSSPAYIAEQEHRKKVLRELNSLISGA

SEQ ID NO: 21 - protein, 464 aa, Solanum lycopersicum
MTDYRLWSNTNTTNTCDDTMMMDSFLSSDPSSFWPASTPNRPTPVNGVGETMPFFNQESLQQRLQALIDGARESWAYAIFWQSSVVDFASQTVLGWGDGYYKGEEDKNKRRGSSSSAANFVAEQEHRKKVLRELNSLISGVQASAGNGTDDAVDEEVTDTEWFFLISMTQSFVNGNGLPGLAMYSSSPIWVTGTEKLAASQCERARQAQGFGLQTIVCIPSPESREILNFGDSSKRFSGQSQLGPGPGLMEENKNKNKNKKRSLGSRGNNEEGMLSFVSGVILPTSTMGKSGDSDHSDLEASVVKEAVVEPEKKPRKRGRKPANGREEPLNHVEAERQRREKLNQRFYELRSQIECLRKELTNKGSSNYSASPPLNQDVKIVDMDIDVKVIGWDAMIRIQCSKKNHPAARLMAALKDLDLDVHHASVSVVNDLMIQQATVKMGSRLYAQEQLRIALTSKIAESR

SEQ ID NO: 22 - protein, 54 aa, Solanum lycopersicum
FASQTVLGWGDGYYKGEEDKNKRRGSSSSAANFVAEQEHRKKVLRELNSLISGV

SEQ ID NO: 23 - protein, 692 aa, Solanum tuberosum
MTEYSLPTMNLWNNSTSDDNVSMMEAFMSSDLSFWATTNSTTTNSASAAVVGVNSNLLHTNNNNPSVFPLSSSTSVSAAAAVDATKSMPFFNQETLQQRLQALIDGARETWTYAIFWQSSVVDFSSPSVLGWGDGYYKGEEDKAKRKLAVSSPAYIAEQEHRKKVLRELNSLISGAPAGTDDAVDEEVTDTEWFFLISMTQSFVNGSGLPGQALYSSSPIWVAGTEKLAASHCERVRQAQGFGLQTIVCIPSANGVVELGSTELIVESSDLMNKVRVLFNFSNDLGSGSWAVQPESDPSALWLTEPSSSGMEVRESLNTVQTNSVPSSNSNKQIAYANENNHQSGNGQSCYNLQQQQNNPPQQQTQGFFTRELNFSEFGFDGSSNRNGNASLSCKPESGEILNFGDSTKKSASSANVNLFTGQSQFGAVEENNNNKNKKRSATSRGSNEEGMLSFVSGTVLPSSGMKSGGGGGEDSEHSDLEASVVKEADSSRVVEPEKRPRKRGRKPANGREEPLNHVEAERQRREKLNQRFYALRAVVPNVSKMDKASLLGDAISYINELKSKLQNTESDKEDLKSQIEDLKKESRRPGPPPPNQDLKIGGKIVDVDIDVKIIGWDAMIGIQCNKKNHPAARLMAALMELDLDVHHASVSVVNDLMIQQATVKMGSRHYTEEQLRVALKSKIAETPLESR

SEQ ID NO: 24 - protein, 53 aa, Solanum tuberosum
FSSPSVLGWGDGYYKGEEDKAKRKLAVSSPAYIAEQEHRKKVLRELNSLISGA

SEQ ID NO: 25 - protein, 646 aa, Solanum tuberosum
MTDYRLWSNSNTTNTSDDNMMMDAFLSSDPSSFWPNRTSISPTPVNGGVGETMPFFNQESLQQRLQALIDGARESWAYAIFWQSSSTSDFATPSVLGWGDGYYKGEENKNKRRASSSSTNFVAEQEHRKKVLRELNSLISGVQATGAGSGGDDAVDEEVTDTEWFFLISMTQSFANGNGLPGLAMYSSSPIWVTGTEKLAGSQCERARQAQGFGLQTIVCIPSANGVVELGSTELIFESSDLMNKVKYLFNFNIDMGSVTGSGSGSCAVHPEPDPSALWLTDPSSSVVEAKDSLINSSSRDVQLVFGNENSENGTQNQQHSQQTQGFFTKELNFSGYGFDGSSTRNKNGNSSISCKPETREILNFGDSSKKSGSLFSGQSQFGPGTGLGLMEENKNNNKKRSLASRGNNEKGMLSFVSGVILPTSTMGKSGGGGNFDHSDLEASVVKEAIVEPERKPRKRGRKPANGREEPLNHVEAERQRREKLNQRFYALRAVVPNVSKMDKASLLGDAIAYINELKSKVQNSDLDKEELRSQIESLRKELANKGSSNYSSSPPSNQDLKIVDMDIDVKVIGWDAMIRIQCSKKNHPAARLMAALKDLDLDVHHASVSVVNDLMIQQATVKMGSRLYAQEQLTIALTSKFAESR

SEQ ID NO: 26 - protein, 53 aa, Solanum tuberosum
FATPSVLGWGDGYYKGEENKNKRRASSSSTNFVAEQEHRKKVLRELNSLISGV

SEQ ID NO: 27 - protein, 699 aa, Catharanthus roseus
MTDYRLQPKMNLWGTTTNTAASPIITSDDNSSMMEAFMTSSDPISLWPPSMSVNHHHPPTPTSSAVTTAVDSAKSMPAQPAFFNQENLQQRLQTLIDGARESWTYAIFWQSSVVEFAGPSVLGWGDGYYKGEEDKGKRKNSSSASSFAEQEHRKKVLRELNSLIAGPQGTADDAVDEEVTDTEWFFLISMTQSFVSGSGLPGQALYNSNPVWVTGAGRLAVSHCDRARQAQSFGLQTLVCIPSANGVVELGSTELIFQSSDLMNKVRILFNFNNIDLGSSSGPWPENDPSSLWLTDPSPSGVGVKEGVNTNNNTSVQGNSIPSGNKQQLVFGNNDNHPTTSTLTDHPGAGAVNSYNNSSQNAQQPQGSFFTRELNFSEYGFERSSVKNGNCKPESGEILNFGGESVTKKNSVSGNGNLFSVQSQFGAGEENKNKKRPSPVSRGSNDEGMLSFTSGVVLPSTGVVKSSGGGGGGDSDHSDLEASVVKEAESSRVVDPEKRPRKRGRKPANGREEPLNHVEAERQRREKLNQRFYALRAVVPNVSKMDKASLLGDAISYINELKAKLQTTETDKDELKNQLDSLKKELASKESRLLSSPDQDLKSSNKQSVGNLDMDIDVKIIGREAMIRVQSSKNNHPAARVMGALKDLDLELLHASVSVVNDLMIQQNTVRMGSRFYTQEQLRIALTSRIAGNSMRLLV

SEQ ID NO: 28 - protein, 51 aa, Catharanthus roseus
FAGPSVLGWGDGYYKGEEDKGKRKNSSSASSFAEQEHRKKVLRELNSLIAG

SEQ ID NO: 29 - skipped

SEQ ID NO: 30 - protein, 1172 aa, Arabidopsis thaliana
MVSGVGGSGGGRGGGRGGEEEPSSSHTPNNRRGGEQAQSSGTKSLRPRSNTESMSKAIQQYTVDARLHAVFEQSGESGKSFDYSQSLKTTTYGSSVPEQQITAYLSRIQRGGYIQPFGCMIAVDESSFRIIGYSENAREMLGIMPQSVPTLEKPEILAMGTDVRSLFTSSSSILLERAFVAREITLLNPVWIHSKNTGKPFYAILHRIDVGVVIDLEPARTEDPALSIAGAVQSQKLAVRAISQLQALPGGDIKLLCDTVVESVRDLTGYDRVMVYKFHEDEHGEVVAESKRDDLEPYIGLHYPATDIPQASRFLFKQNRVRMIVDCNATPVLVVQDDRLTQSMCLVGSTLRAPHGCHSQYMANMGSIASLAMAVIINGNEDDGSNVASGRSSMRLWGLVVCHHTSSRCIPFPLRYACEFLMQAFGLQLNMELQLALQMSEKRVLRTQTLLCDMLLRDSPAGIVTQSPSIMDLVKCDGAAFLYHGKYYPLGVAPSEVQIKDVVEWLLANHADSTGLSTDSLGDAGYPGAAALGDAVCGMAVAYITKRDFLFWFRSHTAKEIKWGGAKHHPEDKDDGQRMHPRSSFQAFLEVVKSRSQPWETAEMDAIHSLQLILRDSFKESEAAMNSKVVDGVVQPCRDMAGEQGIDELGAVAREMVRLIETATVPIFAVDAGGCINGWNAKIAELTGLSVEEAMGKSLVSDLIYKENEATVNKLLSRALRGDEEKNVEVKLKTFSPELQGKAVFVVVNACSSKDYLNNIVGVCFVGQDVTSQKIVMDKFINIQGDYKAIVHSPNPLIPPIFAADENTCCLEWNMAMEKLTGWSRSEVIGKMIVGEVFGSCCMLKGPDALTKFMIVLHNAIGGQDTDKFPFPFFDRNGKFVQALLTANKRVSLEGKVIGAFCFLQIPSPELQQALAVQRRQDTECFTKAKELAYICQVIKNPLSGMRFANSLLEATDLNEDQKQLLETSVSCEKQISRIVGDMDLESIEDGSFVLKREEFFLGSVINAIVSQAMFLLRDRGLQLIRDIPEEIKSIEVFGDQIRIQQLLAEFLLSIIRYAPSQEWVEIHLSQLSKQMADGFAAIRTEFRMACPGEGLPPELVRDMFHSSRWTSPEGLGLSVCRKILKLMNGEVQYIRESERSYFLIILELPVPRKRPLSTASGSGDMMLMMPY

SEQ ID NO: 31 - DNA, 4550 bp, Arabidopsis thaliana
cttcaatttattttattggtttctccacttatctccgatctcaattctccccattttcttcttcctcaagttcaaaattcttgagaatttagctctaccagaattcgtctccgataactagtggatgatgattcaccctaaatccttccttgtctcaaggtaattctgagaaatttctcaaattcaaaatcaaacggcatggtttccggagtcgggggtagtggcggtggccgtggcggtggccgtggcggagaagaagaaccgtcgtcaagtcacactcctaataaccgaagaggaggagaacaagctcaatcgtcgggaacgaaatctctcagaccaagaagcaacactgaatcaatgagcaaagcaattcaacagtacaccgtcgacgcaagactccacgccgttttcgaacaatccggcgaatcagggaaatcattcgactactcacaatcactcaaaacgacgacgtacggttcctctgtacctgagcaacagatcacagcttatctctctcgaatccagcgaggtggttacattcagcctttcggatgtatgatcgccgtcgatgaatccagtttccggatcatcggttacagtgaaaacgccagagaaatgttagggattatgcctcaatctgttcctactcttgagaaacctgagattctagctatgggaactgatgtgagatctttgttcacttcttcgagctcgattctactcgagcgtgctttcgttgctcgagagattaccttgttaaatccggtttggatccattccaagaatactggtaaaccgttttacgccattcttcataggattgatgttggtgttgttattgatttagagccagctagaactgaagatcctgcgctttctattgctggtgctgttcaatcgcagaaactcgcggttcgtgcgatttctcagttacaggctcttcctggtggagatattaagcttttgtgtgacactgtcgtggaaagtgtgagggacttgactggttatgatcgtgttatggtttataagtttcatgaagatgagcatggagaagttgtagctgagagtaaacgagatgatttagagccttatattggactgcattatcctgctactgatattcctcaagcgtcaaggttcttgtttaagcagaaccgtgtccgaatgatagtagattgcaatgccacacctgttcttgtggtccaggacgataggctaactcagtctatgtgcttggttggttctactcttagggctcctcatggttgtcactctcagtatatggctaacatgggatctattgcgtctttagcaatggcggttataatcaatggaaatgaagatgatgggagcaatgtagctagtggaagaagctcgatgaggctttggggtttggttgtttgccatcacacttcttctcgctgcataccgtttccgctaaggtatgcttgtgagtttttgatgcaggctttcggtttacagttaaacatggaattgcagttagctttgcaaatgtcagagaaacgcgttttgagaacgcagacactgttatgtgatatgcttctgcgtgactcgcctgctggaattgttacacagagtcccagtatcatggacttagtgaaatgtgacggtgcagcatttctttaccacgggaagtattacccgttgggtgttgctcctagtgaagttcagataaaagatgttgtggagtggttgcttgcgaatcatgcggattcaaccggattaagcactgatagtttaggcgatgcggggtatcccggtgcagctgcgttaggggatgctgtgtgcggtatggcagttgcatatatcacaaaaagagactttcttttttggtttcgatctcacactgcgaaagaaatcaaatggggaggcgctaagcatcatccggaggataaagatgatgggcaacgaatgcatcctcgttcgtcctttcaggcttttcttgaagttgttaagagccggagtcagccatgggaaactgcggaaatggatgcgattcactcgctccagcttattctgagagactcttttaaagaatctgaggcggctatgaactctaaagttgtggatggtgtggttcagccatgtagggatatggcgggggaacaggggattgatgagttaggtgcagttgcaagagagatggttaggctcattgagactgcaactgttcctatattcgctgtggatgccggaggctgcatcaatggatggaacgctaagattgcagagttgacaggtctctcagttgaagaagctatggggaagtctctggtttctgatttaatatacaaagagaatgaagcaactgtcaataagcttctttctcgtgctttgagaggtatattcagttcttcagctatgttgtatctgcggtgtatataccaattcgcgggtatttgattattttgttgcatttggcaatgcaggggacgaggaaaagaatgtggaggttaagctgaaaactttcagccccgaactacaagggaaagcagtttttgtggttgtgaatgcttgttccagcaaggactacttgaacaacattgtcggcgtttgttttgttggacaagacgttactagtcagaaaatcgtaatggataagttcatcaacatacaaggagattacaaggctattgtacatagcccaaaccctctaatcccgccaatttttgctgctgacgagaacacgtgctgcctggaatggaacatggcgatggaaaagcttacgggttggtctcgcagtgaagtgattgggaaaatgattgtcggggaagtgtttgggagctgttgcatgctaaagggtcctgatgctttaaccaagttcatgattgtattgcataatgcgattggtggccaagatacggataagttccctttcccattctttgaccgcaatgggaagtttgttcaggctctattgactgcaaacaagcgggttagcctcgagggaaaggttattggggctttctgtttcttgcaaatcccgagccctgagctgcagcaagctttagcagtccaacggaggcaggacacagagtgtttcacgaaggcaaaagagttggcttatatttgtcaggtgataaagaatcctttgagcggtatgcgtttcgcaaactcattgttggaggccacagacttgaacgaggaccagaagcagttacttgaaacaagtgtttcttgcgagaaacagatctcaaggatcgtcggggacatggatcttgaaagcattgaagacgggtgagtatagttagaatttatctagaagctagttttgcttacttcacaaaatgtgaccaaatcccaaattttgtttttttcattgatcagttcatttgtgctaaagagggaagagtttttccttggaagtgtcataaacgcgattgtaagtcaagcgatgttcttattaagggacagaggtcttcagctgatccgtgacattcccgaagagatcaaatcaatagaggtttttggagaccagataaggattcaacagctcctggctgagtttctgctgagtataatccggtatgcaccatctcaagagtgggtggagatccatttaagccaactttcaaagcaaatggctgatggattcgccgccatccgcacagaattcaggtacatttcattgttcccgctgttgtctccacatatccataaccaaaattatgcaatccggtttttttggttccttattttgtacataaagaaaatgaatttggtttggttaattacgaatttgatttaggcgtttaaagaatttgaggttttaaccaattcactatttgttttggttattgtttagttggaacctagattagtttgatttttgtattcggtttagtcgacttgggaacttttagacacatccataggcctagaattagcagtcaaggaatgtaatgttttcaaattgatgaaaaccagctcaaaagtgtaaaacttgggtttcatgtgttggtgtctttgttatgtctttattcgttgtttgcagaatggcgtgtccaggtgaaggtctgcctccagagctagtccgagacatgttccatagcagcaggtggacaagccctgaaggtttaggtctaagcgtatgtcgaaagattttaaagctaatgaacggtgaggttcaatacatccgagaatcagaacggtcctatttcctcatcattctggaactccctgtacctcgaaagcgaccattgtcaactgctagtggaagtggtgacatgatgctgatgatgccatattagtcacacttcagttggtatgagagtttgtatcattgtatgagtgtttgtgtgtctaacgacgtcggaggaggatagaaagttttttttttgtttccggtgagattagtagagaagagggagattatttgcgttcagctcagctcgccggaaaaaaaacgtaacagtagttgtagagaatttcaagacttttgtttgtgctgtgtaaattgacaactccgagagaaacaaaacaatgagataagaagagagcatattaatcgatgaccaatccttttaatt

SEQ ID NO: 32 - protein, 1161 aa, Zea mays
MASGSRATPTRSPSSARPEAPRHAHHHHHSQSSGGSTSRAGGGAAATESVSKAVAQYTLDARLHAVFEQSGASGRSFDYSQSLRAPPTPSSEQQIAAYLSRIQRGGHIQPFGCTLAVADDSSFRLLAFSENSPDLLDLSPHHSVPSLDSSAPPHVSLGADARLLFSPSSAVLLERAFAAREISLLNPIWIHSRVSSKPFYAILHRIDVGVVIDLEPARTEDPALSIAGAVQSQKLAVRAISRLQALPGGDVKLLCDTVVEHVRELTGYDRVMVYRFHEDEHGEVVAESRRDNLEPYLGLHYPATDIPQASRFLFRQNRVRMIADCHATPVRVIQDPGLSQPLCLVGSTLRAPHGCHAQYMANMGSIASLVMAVIISSGGDDEQTGRGGISSAMKLWGLVVCHHTSPRCIPFPLRYACEFLMQAFGLQLNMELQLAHQLSEKHILRTQTLLCDMLLRDSPTGIVTQSPSIMDLVKCDGAALYYHGKYYPLGVTPTESQIKDIIEWLTVFHGDSTGLSTDSLADAGYLGAAALGEAVCGMAVAYITPSDYLFWFRSHTAKEIKWGGAKHHPEDKDDGQRMHPRSSFKAFLEVVKSRSLPWENAEMDAIHSLQLILRDSFRDAAEGTNNSKAIVNGQVQLRELELRGINELSSVAREMVRLIETATVPIFAVDTDGCINGWNAKIAELTGLSVEEAMGKSLVNDLIFKESEATVEKLLSRALRGEEDKNVEIKLKTFGSEQSKGPIFVVVNACSSRDYTQNIVGVCFVGQDVTGQKVVMDKFVNIQGDYKAIVHNPNPLIPPIFASDENTSCSEWNTAMEKLTGWSRGEVVGKFLIGEVFGNCCRLKGPDALTKFMVIIHNAIGGQDYEKFPFSFFDKNGKYVQALLTANTRSKMDGKSIGAFCFLQIASTEIQQAFEIQRQQEKKCYARMKELAYICQEIKNPLSGIRFTNSLLQMTDLNDDQRQFLETSSACEKQMSKIVKDASLQSIEDGSLVLEQSEFSLGDVMNAVVSQAMLLLRERDLQLIRDIPDEIKDASAYGDQCRIQQVLADFLLSMVRSAPSENGWVEIQVRPNVKQNSDGTNTELFIFRFACPGEGLPADVVQDMFSNSQWSTQEGVGLSTCRKILKLMGGEVQYIRESERSFFLIVLEQPQPRPAAGREIV

SEQ ID NO: 33 - protein, 1161 aa, Zea mays
MASGSRATPTRSPSSARPEAPRHAHHHHHSQSSGGSTSRAGGGAAATESVSKAVAQYTLDARLHAVFEQSGASGRSFDYSQSLRAPPTPSSEQQIAAYLSRIQRGGHIQPFGCTLAVADDSSFRLLAFSENSPDLLDLSPHHSVPSLDSSAPPHVSLGADARLLFSPSSAVLLERAFAAREISLLNPIWIHSRVSSKPFYAILHRIDVGVVIDLEPARTEDPALSIAGAVQSQKLAVRAISRLQALPGGDVKLLCDTVVEHVRELTGYDRVMVYRFHEDEHGEVVAESRRDNLEPYLGLHYPATDIPQASRFLFRQNRVRMIADCHATPVRVIQDPGLSQPLCLVGSTLRAPHGCHAQYMANMGSIASLVMAVIISSGGDDEQTGRGGISSAMKLWGLVVCHHTSPRCIPFPLRYACEFLMQAFGLQLNMELQLAHQLSEKHILRTQTLLCDMLLRDSPTGIVTQSPSIMDLVKCDGAALYYHGKYYPLGVTPTESQIKDIIEWLTVFHGDSTGLSTDSLADAGYLGAAALGEAVCGMAVAYITPSDYLFWFRSHTAKEIKWGGAKHHPEDKDDGQRMHPRSSFKAFLEVVKSRSLPWENAEMDAIHSLQLILRDSFRDAAEGTNNSKAIVNGQVQLRELELRGINELSSVAREMVRLIETATVPIFAVDTDGCINGWNAKIAELTGLSVEEAMGKSLVNDLIFKESEATVEKLLSRALRGEEDKNVEIKLKTFGSEQYKGPIFVVVNACSSRDYTQNIVGVCFVGQDVTGQKVVMDKFVNIQGDYKAIVHNPNPLIPPIFASDENTSCSEWNTAMEKLTGWSRGEVVGKFLIGEVFGNCCRLKGPDALTKFMVIIHNAIGGQDYEKFPFSFFDKNGKYVQALLTANTRSKMDGKSIGAFCFLQIASTEIQQAFEIQRQQEKKCYARMKELAYICQEIKNPLSGIRFTNSLLQMTDLNDDQRQFLETSSACEKQMSKIVKDASLQSIEDGSLVLEQSEFSLGDVMNAVVSQAMLLLRERDLQLIRDIPDEIKDASAYGDQCRIQQVLADFLLSMVRSAPSENGWVEIQVRPNVKQNSDGTNTELFIFRFACPGEGLPADVVQDMFSNSQWSTQEGVGLSTCRKILKLMGGEVQYIRESERSFFLIVLEQPQPRPAAGREIV

SEQ ID NO: 34 - protein, 1166 aa, Zea mays
MASDSRPPKRSPSARRVAPRHAHHHHSQSSGGSTSRAGAGGGGGGAAATESVSKAVAQYNLDARLHAVFEQSGASGRSFDYSQSLRAPPTPSSEQQIAAYLSRIQRGGHIQPLGCTLAVADDSSFRLLAFSENAADLLDLSPHHSVPSLDSVALPPVSLGADARLYFSPSSAVLLERAFAAREISLLNPLWIHSRASSKPFYAILHRIDVGVVIDLEPARTEDPALSIAGAVQSQKLAVRAISRLQALPGGDVKLLCDTVVEHVRELTGYDRVMVYKFHEDEHGEVVAESRRDNLEPYLGLHYPATDIPQASRFLFQQNRVRMIADCHAIPVRVIQDPGLSQQLCLVGSTLRAPHGCHAQYMANMGSIASLVMAVIISSGGDDERTGRGAISSSMKLWGLVVCHHTSPRCIPFPLRYACEFLMQAFGLQLNMELQLAHQLSEKHILRTQTLLCDMLLRDSPAGIITQSPSVMDLVKCDGAALYYRGKYYPLGVTPTESQIKDIIEWLTVCHGDSTGLSTDSLADAGYLGAVALGDAVCGMAVAYITPSDYLFWFRSHTAKEIKWGGAKHHPEDKDDGQRMHPRSSFKAFLEVVKSRSLSWENAEMDAIHSLQLILRDSFRDAAEGTSNSKAIVNGQRQLGELELRGINELSSVAREMVRLIETATVPIFAVDTDGCINGWNAKIAELTGLSVEEAMGKSLVNDLIFKECDDIVEKLLSRALRGEEDKNVEIKLKTFGSEQSKGAIFVIVNACSSRDYTQNIVGVCFVGQDVTGQKVVMDKFINIQGDYKAIVHNPNPLLPPIFASDENTSCSEWNTAMEKLTGWSREEVVGKFLIGEVFGNCCRLKGPDALTKFMVVIHNAIEGHDSEKFPFSFFDKNGKYVQALLTANTRSKMDGKSIGAFCFLQIASAEIQQAFEIQRQQEKKCYARMKELAYICQEIKNPLSGIRFTNSLLQMTDLNDDQRQFLETSSACEKQMSKIVKDASLKSIEDGSLVLEKSEFSLGDVMNAVVSQTMSLLRERDLQLIRDIPDEIKDASAYGDQFRIQQVLADFLLSMAQSAPSENGWVEIQVRPNVKQNYDGTDTELFIFRFACPGEGLPADIVQDMFSNSQWSTQEGVGLSTCRKILKLMGGEVQYIRESERSFFLIVLELPQPRLAAGRENQLIC

SEQ ID NO: 35 - protein, 1137 aa, Glycine max
MASASGAANSSVPPPQIHTSRTKLSHHSSNNNNNIDSMSKAIAQYTEDARLHAVFEQSGESGRSFNYSESIRIASESVPEQQITAYLVKIQRGGFIQPFGSMIAVDEPSFRILGYSDNARDMLGITPQSVPSLDDKNDAAFALGTDVRALFTHSSALLLEKAFSAREISLMNPIWIHSRTSGKPFYGILHRIDVGIVIDLEPARTEDPALSIAGAVQSQKLAVRAISQLQSLPGGDVKLLCDTVVESVRELTGYDRVMVYKFHEDEHGEVVSESKRPDLEPYIGLHYPATDIPQASRFLFKQNRVRMIVDCHASAVRVVQDEALVQPLCLVGSTLRAPHGCHAQYMANMGSIASLVMAVIINGNDEEGVGGRSSMRLWGLVVCHHTSARCIPFPLRYACEFLMQAFGLQLNMELQLAAQSLEKRVLRTQTLLCDMLLRDSPTGIVTQSPSIMDLVKCDGAALYFQGNYYPLGVTPTEAQIRDIIEWLLAFHGDSTGLSTDSLGDAGYPGAASLGDAVCGMAVAYITEKDFLFWFRSHTAKEIKWGGAKHHPEDKDDGQRMHPRSSFKAFLEVVKSRSLPWENAEMDAIHSLQLILRDSFKDAEHRNSKAVVDPHVSEQELQGVDELSSVAREMVRLIETATAPIFAVDVDGHVNGWNAKVSELTGLPVEEAMGKSLVHDLVFKESEETMNKLLSRALKGEEDKNVEIKMRTFGPEHQNKAVFLVVNACSSKDFTNNVVGVCFVGQDVTGQKIVMDKFINIQGDYKAIVHSPNPLIPPIFASDDNTCCLEWNTAMEKLTGWGRVDVIGKMLVGEVFGSCCQLKGSDSITKFMIVLHNALGGQDTDKFPFSFLDRHGKYVQTFLTANKRVNMEGQIIGAFCFLQIMSPELQQALKAQRQQEKNSFGRMKELAYICQGVKNPLSGIRFTNSLLEATSLTNEQKQFLETSVACEKQMLKIIRDVDLESIEDGSLELEKGEFLLGNVINAVVSQVMLLLRERNLQLIRDIPEEIKTLAVYGDQLRIQQVLSDFLLNIVRYAPSPDGWVEIHVRPRIKQISDGLTLLHAEFRMVCPGEGLPPELIQDMFNNSRWGTQEGLGLSMSRKILKLMNGEVQYIREAERCYFYVLLELPVTRRSSKKC

SEQ ID NO: 36 - protein, 1100 aa, Glycine max
MSKAIAQYTEDARLHAVFEQSGESGRSFNYSESIRIASESVPEQQITAYLVKIQRGGFIQPFGSMIAVDEPSFRILGYSDNARDMLGITPQSVPSLDDKNDAAFALGTDVRALFTHSSALLLEKAFSAREISLMNPIWIHSRTSGKPFYGILHRIDVGIVIDLEPARTEDPALSIAGAVQSQKLAVRAISQLQSLPGGDVKLLCDTVVESVRELTGYDRVMVYKFHEDEHGEVVSESKRPDLEPYIGLHYPATDIPQASRFLFKQNRVRMIVDCHASAVRVVQDEALVQPLCLVGSTLRAPHGCHAQYMANMGSIASLVMAVIINGNDEEGVGGRSSMRLWGLVVCHHTSARCIPFPLRYACEFLMQAFGLQLNMELQLAAQSLEKRVLRTQTLLCDMLLRDSPTGIVTQSPSIMDLVKCDGAALYFQGNYYPLGVTPTEAQIRDIIEWLLAFHGDSTGLSTDSLGDAGYPGAASLGDAVCGMAVAYITEKDFLFWFRSHTAKEIKWGGAKHHPEDKDDGQRMHPRSSFKAFLEVVKSRSLPWENAEMDAIHSLQLILRDSFKDAEHRNSKAVVDPHVSEQELQGVDELSSVAREMVRLIETATAPIFAVDVDGHVNGWNAKVSELTGLPVEEAMGKSLVHDLVFKESEETMNKLLSRALKGEEDKNVEIKMRTFGPEHQNKAVFLVVNACSSKDFTNNVVGVCFVGQDVTGQKIVMDKFINIQGDYKAIVHSPNPLIPPIFASDDNTCCLEWNTAMEKLTGWGRVDVIGKMLVGEVFGSCCQLKGSDSITKFMIVLHNALGGQDTDKFPFSFLDRHGKYVQTFLTANKRVNMEGQIIGAFCFLQIMSPELQQALKAQRQQEKNSFGRMKELAYICQGVKNPLSGIRFTNSLLEATSLTNEQKQFLETSVACEKQMLKIIRDVDLESIEDGSLELEKGEFLLGNVINAVVSQVMLLLRERNLQLIRDIPEEIKTLAVYGDQLRIQQVLSDFLLNIVRYAPSPDGWVEIHVRPRIKQISDGLTLLHAEFRMVCPGEGLPPELIQDMFNNSRWGTQEGLGLSMSRKILKLMNGEVQYIREAERCYFYVLLELPVTRRSSKKC

SEQ ID NO: 37 - protein, 1171 aa, Oryza sativa
MASGSRATPTRSPSSARPAAPRHQHHHSQSSGGSTSRAGGGGGGGGGGGGGAAAAESVSKAVAQYTLDARLHAVFEQSGASGRSFDYTQSLRASPTPSSEQQIAAYLSRIQRGGHIQPFGCTLAVADDSSFRLLAYSENTADLLDLSPHHSVPSLDSSAVPPPVSLGADARLLFAPSSAVLLERAFAAREISLLNPLWIHSRVSSKPFYAILHRIDVGVVIDLEPARTEDPALSIAGAVQSQKLAVRAISRLQALPGGDVKLLCDTVVEHVRELTGYDRVMVYRFHEDEHGEVVAESRRNNLEPYIGLHYPATDIPQASRFLFRQNRVRMIADCHAAPVRVIQDPALTQPLCLVGSTLRSPHGCHAQYMANMGSIASLVMAVIISSGGDDDHNIARGSIPSAMKLWGLVVCHHTSPRCIPFPLRYACEFLMQAFGLQLNMELQLAHQLSEKHILRTQTLLCDMLLRDSPTGIVTQSPSIMDLVKCDGAALYYHGKYYPLGVTPTEVQIKDIIEWLTMCHGDSTGLSTDSLADAGYPGAAALGDAVSGMAVAYITPSDYLFWFRSHTAKEIKWGGAKHHPEDKDDGQRMHPRSSFKAFLEVVKSRSLPWENAEMDAIHSLQLILRDSFRDSAEGTSNSKAIVNGQVQLGELELRGIDELSSVAREMVRLIETATVPIFAVDTDGCINGWNAKVAELTGLSVEEAMGKSLVNDLIFKESEETVNKLLSRALRGDEDKNVEIKLKTFGPEQSKGPIFVIVNACSSRDYTKNIVGVCFVGQDVTGQKVVMDKFINIQGDYKAIVHNPNPLIPPIFASDENTCCSEWNTAMEKLTGWSRGEVVGKLLVGEVFGNCCRLKGPDALTKFMIVLHNAIGGQDCEKFPFSFFDKNGKYVQALLTANTRSRMDGEAIGAFCFLQIASPELQQAFEIQRHHEKKCYARMKELAYIYQEIKNPLNGIRFTNSLLEMTDLKDDQRQFLETSTACEKQMSKIVKDASLQSIEDGSLVLEKGEFSLGSVMNAVVSQVMIQLRERDLQLIRDIPDEIKEASAYGDQYRIQQVLCDFLLSMVRFAPAENGWVEIQVRPNIKQNSDGTDTMLFLFRFACPGEGLPPEIVQDMFSNSRWTTQEGIGLSICRKILKLMGGEVQYIRESERSFFHIVLELPQPQQAASRGTS

SEQ ID NO: 38 - protein, 428 aa, Arabidopsis thaliana
MEHQGWSFEENYSLSTNRRSIRPQDELVELLWRDGQVVLQSQTHREQTQTQKQDHHEEALRSSTFLEDQETVSWIQYPPDEDPFEPDDFSSHFFSTMDPLQRPTSETVKPKSSPEPPQVMVKPKACPDPPPQVMPPPKFRLTNSSSGIRETEMEQYSVTTVGPSHCGSNPSQNDLDVSMSHDRSKNIEEKLNPNASSSSGGSSGCSFGKDIKEMASGRCITTDRKRKRINHTDESVSLSDAIGNKSNQRSGSNRRSRAAEVHNLSERRRRDRINERMKALQELIPHCSKTDKASILDEAIDYLKSLQLQLQVMWMGSGMAAAAASAPMMFPGVQPQQFIRQIQSPVQLPRFPVMDQSAIQNNPGLVCQNPVQNQIISDRFARYIGGFPHMQAATQPMEMLRFSSPAGQQSQQPSSVPTKTTDGSRLDH

SEQ ID NO: 39 - DNA, 1747 bp, Arabidopsis thaliana
actttctgtctgtacccaaaagaagtaatgaacctctctcatcttcttcttctctgtttctttcatgttttgtgagttgtttctcaacaattttctggtctcttagagtgagaggagagagatagagagttgtgttgggcgtggaacttggactagttccacatatcaggttatatagatcttctctttcaacttctgattcgtccagaagctttcctaatctgagatctgacatggaacaccaaggttggagttttgaggagaattatagtttgtccactaatagaagatctatcaggccacaagatgaactagtggagttattatggcgagatggacaagtggttctgcagagccaaactcatagagaacaaacccaaacccagaaacaagatcatcatgaagaagccctaagatccagcacctttcttgaagatcaagaaactgtctcttggatccaataccctccagatgaagacccattcgaacccgacgacttctcctcccacttcttctcaaccatggatcccctccagagaccaacctcagagacggttaagcctaagtccagtcctgaacctcctcaagtcatggttaagcctaaggcctgtcctgaccctcctcctcaagtcatgcctcctccaaaatttaggttaacaaattcatcatcggggattagggaaacagaaatggaacagtactcggtaacgaccgttggacctagccattgcggaagcaacccatcacagaacgatctcgatgtctcaatgagtcatgatcgaagcaaaaacatagaagaaaagcttaatccgaacgcaagttcctcatcaggtggctcctctggttgcagctttggcaaagatatcaaagaaatggctagtggaagatgcatcacaaccgaccgtaagagaaaacgtataaatcacactgacgaatctgtatctctatcagatgcaatcggtaacaagtcgaaccaacgatcaggatcaaaccgaaggagtcgagcagctgaagttcataatctctccgaaaggaggaggagagataggatcaatgagagaatgaaggctttgcaagaactaatacctcactgcagtaaaactgataaagcttcgattttagacgaagccatagattatttgaaatcacttcagttacagcttcaagtgatgtggatggggagtggaatggcggcggcggcggcttcggctccgatgatgttccccggagttcaacctcagcagttcatacgtcagatacagagcccggtacagttacctcgatttccggttatggatcagtctgcaattcagaacaatcccggtttagtttgccaaaacccggtacaaaaccagatcatctccgaccggtttgctagatacatcggtgggttcccacacatgcaggccgcgactcagccgatggagatgttgagatttagttcaccggcgggacagcaaagtcaacaaccgtcgtctgtgccgacgaagaccaccgacggttctcgtttggaccactaggttggtgagccacttttttacttccttatttttggtatgtttcttttttatatctatctttctgaacatacttaaaacgttcaaggatgtattattatagagtaaacgtgcaacttcattacgttattttctgtatatgtgagtttatgtatgtcaaaatgacatgatgagattttttgtaaacaacatcttaaaaacaggacatgtgatttttgtaatcgtaaaaa

SEQ ID NO: 40 - protein, 397 aa, Zea mays
MQTAIEHACSVVECAATARAAMDMSHYIPDWSSSMGDTFAPLGGEDDDGLIELMWRNGHVVMQAQAPRKPPRPDDDEAAAAQAQAWFQYPVEERADLFSELFGEAQAAVGGARGEAARQSIRMMPPPPPPPRPAQAPREEKACPGDGGTATATDGAGSSVLTVVSSLCGSNGNHVQATAPGDVARARDVLMVTSSSTTRSRSCTTKSEQPGPGPGAARRSGKRKHNDATDAEDVGLECEPAQRTTTAKRRRAAQVHNLSERRRRDRINEKMKALQELIPHCNKADKASMLDEAIEYLKSLQLQLQVVWMGGGIAAAGVHQRTMVAAPGRPPHVASLPASAPDLYTRYLAVDHLPPPPLVPPPRTAAAMGLYPRQNPVPATSSPSFRTTENTRKLWQA

SEQ ID NO: 41 - DNA, 1492 bp, Zea mays
ccttgccctgctgcaacttgaacctcctggcagctcctgtttcaggcaggcagcaagtagggaagaggctctgcagatcagttccatgcagacagcgatcgagcacgcctgctcggtggtggaatgcgctgcgacagcccgagccgccatggacatgagccactacatccccgattggagcagcagcatgggagacaccttcgcgccactgggcggcgaggacgacgacgggctcatcgagctcatgtggcgcaacggccacgtggtcatgcaggcccaggcgccgcggaagccgccgagacccgacgacgacgaggcggcggcggcgcaggcgcaggcgtggttccagtacccggtggaggagagggccgacctcttctcggagctcttcggggaggcgcaggcggccgtcggcggcgcgcgcggggaggccgcgcgccagagtatccggatgatgccgccgccgccgccgccgccgaggcccgcgcaagcgccgcgggaggagaaggcgtgcccgggagacggcggcacggcgacggcgacggacggcgccggctcgtccgtgctcacggtcgtgtccagcctctgcgggagcaacggcaaccacgtgcaggcgacggcgccgggggacgtcgccagggcccgcgacgtgctgatggtgacctcgtcgtcgacgacgcgttccaggtcatgcaccaccaagagcgagcagccgggtcccgggcccggcgctgcccgccggagcggcaagaggaagcataacgacgccaccgatgccgaggacgtggggctggagtgcgagccggcgcagaggacgacgactgccaagcggcgccgcgccgcgcaagtccacaacctctcggagcggaggagacgggacaggatcaacgagaagatgaaggccctgcaggaactcataccccactgcaacaaagcggacaaggcgtcgatgctggacgaggcgatcgagtacctcaagtcgctgcagctccagctgcaggtggtgtggatgggcggcggcatcgcggcggcgggggtgcaccagcggacgatggtggccgcgcccgggcgtcctccccacgtggcttccctgccggcgtcggcgcccgacctctatacgcgctacctcgccgtcgaccacctgccgccaccgcccttggtgccaccgccacgcacggcggcggcgatgggcttgtacccgcgccagaaccccgtgccggcgacgtcgtctccttccttccgaacgaccgaaaatacgcgaaaactatggcaagcctgagattcagatccggggtatggtgaccagctgatgggtcatctagctgcatgcatgtgtgtatgtgttggtagtatggttaagccttgacagagacttgtgatcgagaccgagatcgaccgataggccgtcacttcttttttcttccatctttcagtttttggttgataggccggagtgtaatttgaccagtggtcgagatttgtcaagcgacac

SEQ ID NO: 42 - protein, 562 aa, Glycine max
MNNSIPGWDFESDTCLTNQRKLIGPDQELVELLWKNGQVVMHNQTHRKTLGNSSNLRQVQKSDQSVLRSSGPYGNSSNLDQEDAAPWVQFPLEDPLEQDFCSNLLSELPTCEFESYKPIRQLEEEKFAKFFASGTPHHPTTSSSQPLPPNMKPSCIQGLQGNPIPMPAPRFHGPDSSQKIHDFGASRKVLNFPQFSTPRNNVPSAPGITQFREKTTANMSQSEAREYSVITVGSSHCGSNHIPQEQDVSRISSTGVWATTNNNTTLSAEPEAVRDYVQRPICPKSGQGKSEMIELTVTSSSGGSGSTGIGRTCSLSTRDHGQKRKGTEEEALEEQSEDTELKSADGNKASQRTRSSRRNRAAEVHNQSERRRRDRINEKMRTLQQLIPNSNKTDKASMLEEAIEYLKSLQFQLQVMWMGGGMTPVMFPGIQHYMSQMGMGMGAPSLPSIHNPMQLPKVPHDQAMSVLQIPNQNLMCQNPVLGAFNYQNQMQNPCLPEQYARYMGYHLMQNASQPMNVFRYGSQAVQHSQTMIAPGNNSSGPMSGTANIDDADSGKAGSSTFN

SEQ ID NO: 43 - DNA, 2161 bp, Glycine max
gaccccgttttcaactggtcccgtgttccttcatttgatgccacatgtgcagctacccatgtttttctcgctgttgacgagcacaatatataataaataccatttttttcatgccatatttgctctcttctctctttgtactaataacttggatctatgccactgtccttctccttgttaaaaactgtgccacacgtctgtcaccaaactccctaagcagaagaagcacatgttcagagggagttttgtttcatcagtctctagctagcatatatttctagcttctattcaacaagttgcaaaaaacagactttgccttaaccaaaagaaaatctgtttttaccttaactcagacaactcgtttggtgaaccatgaacaacagtattcctggttgggattttgagagtgatacatgtctcaccaaccaaagaaagctcatagggccggaccaagaacttgtagagctcctatggaaaaatgggcaagtagttatgcacaaccaaacacataggaagacacttgggaattcatctaacttgagacaggtgcagaaaagtgatcaatcagtattaaggtctagcggtccctatggaaactcaagcaacttggatcaagaagatgccgccccatgggtccaattcccacttgaggacccattggaacaagatttttgttcaaaccttttatctgaactaccaacttgtgaatttgaatcttacaagccaatcaggcaattggaagaggaaaagtttgccaaattttttgcttccggtaccccccatcatcctacaacttcaagttcacaaccactaccacctaacatgaaaccctcatgtattcagggactccaagggaatcctattcctatgccagctccaagatttcatggtcctgattcatctcagaaaatccatgactttggagcatcacgaaaggttctaaattttcctcagttttcaacaccccgtaataatgttccatcagcacctggtattacacagtttagagagaaaactactgctaacatgtcacaaagtgaggctagagagtactcagtgatcacagttggttcaagtcactgtggcagcaatcacatccctcaggagcaagatgtaagcaggatttcaagcactggtgtttgggccactactaataataatactactttatctgctgagcctgaagctgtcagagattatgtccaaagaccgatttgtcctaagagtggccaaggaaaatcagagatgattgaactaactgtgacttcatcttccggtggctcgggaagtactggtatcggaagaacctgttccctatcaacaagagatcatggccaaaagagaaaagggacagaagaagaagcgttagaggaacaaagtgaggacacagaacttaaatcagctgatggaaacaaggcttctcagcggacgaggtcttccagaaggaaccgtgcagcagaagtgcataatcaatcagaaaggagaagaagagataggatcaacgagaagatgaggacattgcagcaactgatacctaatagtaacaagacagacaaagcatcaatgttagaagaggcaatcgaatacttgaaatcacttcagtttcagcttcaggttatgtggatggggggtggcatgacaccagtgatgttcccaggaattcagcactatatgtcacaaatgggtatgggaatgggtgcaccttctttgccttccattcacaacccgatgcaattgccaaaagtgccacatgatcaagccatgtctgtgcttcagataccaaaccagaatttaatgtgtcaaaatccagttttgggtgcctttaactaccaaaaccagatgcagaacccgtgccttccagaacaatatgcacgttacatgggttaccatcttatgcaaaatgcctctcagcctatgaatgtgttcagatatggttcccaagcagtgcaacacagtcaaacgatgattgcaccaggcaataatagcagcggacccatgagtggaacagctaatattgatgatgctgacagtggcaaagcgggttcttccacctttaattgaatagtgaatagcaataccttaaaattactcaattgggggaattacctaatggagtacgtcaatcctcacaagcaccaatatgtgctccaattttatgtag

SEQ ID NO: 44 - protein, 409 aa, Oryza sativa
MNQFVPDWNTTSMGDGFAPLGEDDGLVELLWCNGHVVMQSQAPRKPPRPEKTTAAAAAAMAEDESASWFQYPVDDVLEKDLFTELFGEMTAAGGGGGDVRRAACKEERGAVAAFQSRMMPPPWPARGKAEFGDVDDVCGVSEVVMAKMDGAAAAETVGESSMLTIGSSICGSNHVQTPPVGNGKAGAGTAGAARRAHDTATVASSSMRSRSCTAKAEPRDVAAAGVGGKRKQRGGAAMESGSPSEDVEFESAAATCSPAQKTTTAKRRRAAEVHNLSERRRRDRINEKMKALQELIPHCNKTDKASMLDEAIEYLKSLQLQLQMMWMGGGMAPPAVMFPAAGVHQYMQRMGAVGMGPPHMASLPRMPPFMAPPPAAVQSSPVVSMADPYARCLAVDHLQPPPPMFRREY

SEQ ID NO: 45 - DNA, 1749 bp, Oryza sativa
gcgagtcctcttcctgccctgccctgccctgccctgcattctttctttctccaccaggggaatccagttcacccccagtgctgcttctgctgctgcttctgcatcatcttgccctgttaaaaagacacagtgcccttgttctttcgcagttgcaactagcatctcctcctctacttgtactcacttcacacctcagctcagctcagctcatctcctgtcatctcagctcaaagagaaagagctgaaggtgtaagctgatcaccaggaagcagaggctttttttcagattacagttatctgaaacaaccaacttcagaatcaatcagcaaaggtagaaacaagacagagctgctgtgcttctgtgattaattagggttgttaatgccatgaaccagttcgtccctgattggaacaccaccagcatgggcgacggctttgcgccattaggcgaagacgacgggctcgtcgagctgctatggtgcaatggccacgtcgtcatgcagagccaggcgccgcggaagccgccgaggccggagaagacgacggcggcggcggcggcggcgatggcggaggatgagtcggcgtcgtggtttcagtacccggtcgacgacgtgcttgagaaggacctgttcaccgagctgttcggcgaaatgacggcggccggcggcggcggcggcgacgtccgcagggcggcgtgcaaggaggagcgcggcgcggtcgccgcgttccagagcaggatgatgccgccgccgtggccggcgagggggaaggcggagttcggtgacgtcgacgacgtgtgcggcgtctcggaggtcgtcatggcgaagatggacggggcggcggcggcggagacggtcggcgagtcatcgatgctgacaatcgggtcgagcatctgcgggagcaaccacgtccagacgccgccggtggggaacgggaaggccggcgccggcaccgccggcgccgccagaagggcgcacgacacggcgacggtggcgtcgtcgtcgatgaggtcgaggtcctgcaccgccaaggccgagccgcgcgacgtcgcagccgccggcgtcggcggcaagcggaagcagcgcggcggcgccgccatggagtccgggagccccagcgaggacgtggagttcgagtccgccgccgcaacgtgctcgccggcgcagaagacgacgacggcgaagcggcggcgcgccgccgaggtgcacaacctctccgagaggaggagaagagataggatcaatgagaagatgaaagcattacaggagctcatacctcactgcaacaaaacggacaaagcatcgatgctggatgaagcgatcgagtatctcaagtcactgcagctccagctacagatgatgtggatgggcggcggaatggcgccgccggcggtgatgttcccggcggccggcgtgcaccagtacatgcagcggatgggcgccgtcgggatgggcccaccacacatggcgtccctgccgaggatgccgccgttcatggcgccgccgcccgccgccgtgcagagctcgccggtggtcagcatggccgacccctacgcccgctgcctcgccgtcgaccacctccagccaccgcctccgatgtttcgacgcgaatactagggaaggaactaatatcaaataatagaaggggtgagccttcgaatcgagatcgtctagcccaccaccttatagagctagccggaaggccctcgagcgtttctcatattttcagtttcctaagagtttttttttt

SEQ ID NO: 46-47 - skipped (2 entries)

SEQ ID NO: 48 - protein, 187 aa, Arabidopsis thaliana
MSLFPCEASNMDSMVQDVKPTNLFPRQPSFSSSSSSLPKEDVLKMTQTTRSVKPESQTAPLTIFYAGQVIVFNDFSAEKAKEVINLASKGTANSLAKNQTDIRSNIATIANQVPHPRKTTTQEPIQSSPTPLTELPIARRASLHRFLEKRKDRVTSKAPYQLCDPAKASSNPQTTGNMSWLGLAAEI

SEQ ID NO: 49 - DNA, 1527 bp, Arabidopsis thaliana
atattggaggtaggaagaagaactctgcaaccaaaccaaccaaccccaaagccaaacaaagttttatagagaccttccatttctccctctcgtgacaaacgcaatttgcagagaagcaacagcaacaacaagaagaagaagaaaaagatttgagattactttgtatcgatttagctattcgagaaactcttgccgtttgaaagttttaattgttaaagatgtcgagttctatggaatgttctgagttcgtcggtagccggagatttactgggaagaagcctagcttctcacagacgtgtagtcgattgagtcagtatctaaaagagaacggtagctttggagatctgagcttaggaatggcatgcaagcctgatgtcaatggtaagaaaccttctctttctcctagatccacttcttttttcgttttctctgttttttatttcttgaatcttgatcttgaaaacttttcaagaaaattttgaatcgatttcaaagaaattagggagagttagtttgctaaattttgacatagaaaatgattggagagagttctaacttttggatcatatatatttgcaggaactttaggcaactcacgtcagccgacaacaaccatgagtttattcccttgtgaagcttctaacatggattccatggttcaagatgttaaaccgacgaatctgtttcctaggcaaccaagcttttcttcctcatcttcctctcttccaaaggaagatgttttgaaaatgacacagactaccagatctgtgaaaccagagtctcaaactgcaccattgactatattctacgccgggcaagtgattgtattcaatgacttttctgctgagaaagccaaagaagtgatcaacttggcgagcaaaggcaccgctaatagcttagccaagaatcaaaccgatatcagaagcaacatcgctactatcgcaaaccaagttcctcatccaagaaaaaccacaacacaagagccaatccaatcctccccaacaccattgacagaacttcctattgctagaagagcttcacttcaccggttcttggagaagagaaaggacagagttacgtcaaaggcaccataccaattatgcgatccagccaaagcgtcttcaaaccctcaaaccacaggcaacatgtcgtggctcggtttagcagctgaaatatgaatgctaaccaccctcaagccgtaccaagaaattcttttgacgacgttgcttcaagacaagatataaaagctcctatcttcatgctttttgatttaagatacaaactactcaatgattaggaaacttcatatatttgtatgtattgattagtgatcaattattgttagtattcgttatagtctgtttttctactagttattgtcgcctgtctaaatccccttgctatgggttatctcaaaattagtttcgtatgtaactaattttgtaagaacaataatttttgttgacgaaccatactatcaaatactctaaattatatcttgataaatctacctatcaggtaagtagg

SEQ ID NO: 50 - protein, 352 aa, Arabidopsis thaliana
MERDFLGLGSKNSPITVKEETSESSRDSAPNRGMNWSFSNKVSASSSQFLSFRPTQEDRHRKSGNYHLPHSGSFMPSSVADVYDSTRKAPYSSVQGVRMFPNSNQHEETNAVSMSMPGFQSHHYAPGGRSFMNNNNNSQPLVGVPIMAPPISILPPPGSIVGTTDIRSSSKPIGSPAQLTIFYAGSVCVYDDISPEKAKAIMLLAGNGSSMPQVFSPPQTHQQVVHHTRASVDSSAMPPSFMPTISYLSPEAGSSTNGLGATKATRGLTSTYHNNQANGSNINCPVPVSCSTNVMAPTVALPLARKASLARFLEKRKERVTSVSPYCLDKKSSTDCRRSMSECISSSLSSAT

SEQ ID NO: 51 - DNA, 3253 bp, Arabidopsis thaliana
gcgatttgttaataaaactagaaattgcggtgaattaacttcattccacgttttttcattttctccctcaaaagtctctgttttttttcctttttccggcgaagctctatttagcttgattccggcgtttaacacgcgttttaatcgaaacagacatttgagatcgaattaattttgtagcgggctgtgtctttattatagatggagagagattttctcgggttgggttcgaaaaattctccgatcactgtcaaggaggaaaccagcgaaagctctagagattcaggttatttattactcttctcaatttttctgattctgattgtttttaaatcgtagatttgtttgattgattaggagttattaggactacttgtagtatggaatttgtttttggatagctgattttatggcttgctcgggaactggaattgtcagtttgttgcttggagcagaacattgtcctttgcttttctcgggagatgtagaatttggatttggaaaaactagtgttcttttccaaagccttgtcttaaacatgctttcggtcggagaaattaacgagaactaatctcaagcttctaacataattaaactcggtaaacttttttttactagagtaaatttttttgttttgtttgaagagtcttataattgagaaatactttattagtttatactaaaaaaaaaacgaatacgtaaaatgttggaaaagaggggatgtatagagactgatacaaaaatgataaaatagagacggttggtagtaggtagaaagattaaatatactcaaaagagtgagttggattagtttataagatgattaacttcttgattgtgtgagttggattagtttatgagattattaaaatattgattgtgtatttgtgttgtgtgttgattaagcggaacttgcgttagaatattgttcaaggtacaatgtggaaataatagttttctcaccacgaggaatataattatttcaactttgttttcttatcagccaaaacgtgccacaccataaaagtagtgcatcaacatgtggtgtggtgtggtggggttaaagtttgaatctctctttaatttaaactattaaaacaaacttaaattattggagtttcgtacaatgactttcaatcaaatgttttagaattagacacggttttcgaaagtggttttccctcgttgaatttgtcaacagtatcagattctacattgttggttactaatcttttccttgaagtaggtgttgaattaatcctctgttgtttatgtaaggagatctcgagacatttatggttaacagttaacactacatgtttgactttaaactgattatcttttattctttttcttttgtagctcccaacagaggaatgaactggtctttctcaaacaaagtatcagcttcttcttctcagtttctatccttcaggccaactcaagaagatagacatagaaagtctggaaattatcatcttcctcactctggttccttcatgccatcatcagtagctgatgtttatgattcaacccgcaaagctccttacagttctgtacaggtatttgtcatcaaaacctatgttaaccaagacccttgtgttttttttatccttcgcaagatagctttaaaagtgagccctgttttatgagcatatagtaattggttttgagtctagtttagcacaagttcatggcaattagtttgtggatctaatcttggtttaatactgattcattttaagtgtaagctaagcttctcatttttgataagttagttcatacaatgcctcacacctactttatggcttgttactctcagggagtgaggatgttccctaattccaatcaacacgaagaaactaacgcagtttccatgtcgatgccgggtttccagtctcatcattatgcaccaggaggaagaagcttcatgaacaataacaataactcacaacctttggtaggagttcctatcatggcacctccaatttcaatccttcctcctccaggttccattgtagggactactgatattaggtacccactagtcatcatatcatacagaaactctttctacattttcatagttgactaaagacttatttttgtcagatcttcttccaagccaataggttcacctgcgcagttgacgatcttttatgccggttcagtttgtgtttacgatgacatatctcctgaaaaggtatctcaatcattttcttccatatatgcatctcttttactcgtaaggtatggtactcatttgctttctttcatttctcaggcaaaggcgataatgttgctagctgggaacggttcctctatgcctcaagtcttttcgccgcctcaaactcatcaacaagtggtccatcatactcgtgcctctgtcgattcttcagctatgcctcctagcttcatgcctacaatatcttatcttagccctgaagctggaagtagcacaaacggactcggagccacaaaagcgacaagaggcttgacgtcaacatatcacaacaaccaagctaatggatccaatattaactgcccagtaccagtttcttgttctaccaatgtaatggctccaacaggtaaaaaacaaagtcagagacctgatactacattcgccatctaacttactagtattttcatggatgtaacttcattctcgttctgtttcttatgcagtggcattacctctggctcgcaaagcatccctggctaggtttttagagaaacgcaaagaaaggtacgcaacacttctttagaatacaccattcaatagtttcttgggctaactctctttctcgctgtgggtttctcagggtcacgagcgtatccccatattgcttagacaagaagtcatcgacagattgtcgcagatcaatgtctgaatgcattagttcttctctcagctctgcaacctaatttcatctacagtaagaaggttgctttagaccactccacatccatatttgcatttcaatggcggtcttttcaatgtctcagttaatttttcctcactcgccacactgagtttctccttagctttatatatacgatagtgtatactttgtttacatgttttttggtggaatggaacttatgagagcatatcagatatgtacttgggaaaattagtagaaactgtttgtttctttttttttaactctgttcttttgtatatatcactgaagctcgcatatgtataattcatgtaatggaattgcatcgcttctgtttccctaagttattt

SEQ ID NO: 52 - protein, 310 aa, Arabidopsis thaliana
MERDFLGLGSKLSPITVKEETNEDSAPSRGMMDWSFSSKVGSGPQFLSFGTSQQETRVNTVNDHLLSSAAMDQNQRTYFSSLQEDRVFPGSSQQDQTTITVSMSEPNYINSFINHQHLGGSPIMAPPVSVFPAPTTIRSSSKPLPPQLTIFYAGSVLVYQDIAPEKAQAIMLLAGNGPHAKPVSQPKPQKLVHHSLPTTDPPTMPPSFLPSISYIVSETRSSGSNGVTGLGPTKTKASLASTRNNQTAAFSMAPTVGLPQTRKASLARFLEKRKERVINVSPYYVDNKSSIDCRTLMSECVSCPPAHHLH

SEQ ID NO: 53 - DNA, 3187 bp, Arabidopsis thaliana
attagaggaatcataaatcggcggtgtgtgtaacttcaactcacgtttttcatttctctccaaagtccttcaattgttactaattctctctgatctctcatttcttctcttctccggtgacattttttttctcccccgcgaaagctaaaccgtttttgtattctcaacgattgataagcctgatggagagagattttctcgggctgggatcaaagttatctccgataactgtgaaggaggaaactaacgaagattcaggtaattcatcttcaacatcttccattatgatctgatgattgtgtttttcatctcacttttttttgtttctatttttgtaatctctttttttgtttattgttcaagtacatatatattgtttttctagcttgattgggagtcctactgtctggttttttcttgaacaagaaattttttcttcgttttctcgggaagagaaaaaataaattagggtttcttttttcttgatatatatttaagaaattaggttttagtactatagacagaaatttagctactcgaatttgtttgacgtagccgatgaaaaaacacgttttgggactcgatagttagaaaattcatacgttcacgatctacttttgaagtttttttcattaaatattttttgcaaactacaaatgtacaagtatacaactatacaagcaaacaccaaacttgttgacgttagtaatttaacaagtgttagtattatctttgaaaaataatattcagagaacaaacttgattttctaggtgactaggtgatgcatgtttctaaagctgttggtaatgttgagtgttttcaaaataatttcgtttttttcttcaaacagccgacaccgacagaacaaaaatgctatattttttttgttgcttacaaaattgatcaattggtttcaatacaatagtatcttctttagaaaagattgtttttttcaaagccggattgaatattgagaattagaacattggctggttattctttttgaaaagtttatgccattttttaaggtttattaagcaacttgaattctatcagtattatttaaaaacgaagacgtgaaatgttgggaaaagaatgcgttatatagcgaccggctgacgattagagatttaacaacaaatgcaagttgaattatataaaagcaagattgattgtgacttgattaagttttatttctatccaagtagactcattgattaagttaggatcatgttgggtattaaatttagatcaagttacaatttggatgaataatttacttacccacgaggaatttaatagttagttcttgtctttttatattccgaaacgtgccatttcttgaaagtatttgtatgatcactattttccccagtgtgtttggctttatgcagatttgttcattgttgatgaatctaatgttaagagtcgtccactttagcatagctagatctgagtgtttcctagtttgataaaatctaaagacatttgctcatgtttcagccccaagtagaggtatgatggattggtcattctcaagcaaagtcggttctggtcctcagtttctttcttttgggacatcccaacaagaaacgcgtgtaaacacagtcaatgatcatttgctttcttctgctgcaatggatcaaaaccagagaacttacttcagctcactacaggttaggctatttcttgaaaagaaaaaaagtagtgataaagtgtgatttagtgaccttgtaagaaagcttggcaattggtttagtttcttctggtctcaaaattgatacaaaatgatctcaggaagacagagtgttcccaggttccagtcagcaagaccaaacaaccatcacagtctccatgtccgaaccaaactacatcaacagtttcataaaccaccaacatttaggaggatctcctatcatggcacctccagtttcagtatttcctgctccaaccactattaggcatgcactgcattctatcttcttctgtttaacatcagatacagaacctctttacttctatagttgactcgagctcctttatgttcatctccagatcttcttcaaaaccacttccccctcagttgacaatcttttatgccggttcagtattagtttaccaagacatagctcctgaaaaggtaaccaaatttccttcaatatgtgttacattacagtccaagctatccactgactaagtattcaatcaaagaaataagtttcacgtatagacatgctgaagttatagaaagttactaacctggtttcaacatacagtatgttaatgattcatagatatgataaatctttgtccttacttcttcatttattttgtattcataggcccaagctatcatgttgctagccggaaatggacctcatgctaaaccggtttcacaacctaaacctcaaaaactggttcatcactctcttccaaccactgatcctccaactatgcctcctagtttcctgccttccatctcttacattgtctctgaaaccagaagtagtggatccaacggggttactggacttggaccaacaaaaacaaaggcgagtttagcatccacgcgcaacaaccaaactgctgccttctctatggctccaacaggttataaatgaagtcttaactcctattaatgttttgtcatcaaacttctatcttaggtttagtttgttataaccaaaaaatcttgctatgatttaatacagtgggtttaccacaaacacgcaaagcatccttggctcggttcttagagaaacgcaaagaaaggtactgagctacaagattattcacttattcacaatatcaaaacacaggtttgctgtatattggcttcgttttcttgcagggtcattaacgtatcaccttattacgtagacaacaagtcatcaatagactgtagaacactgatgtctgaatgtgtaagctgtcctccagctcatcatctgcactaaaaccaatttagacccctcattgttctaaaggctttttcttttttctctggctctgtatcctatagactatagtatagttgttatagcttttgtttattcagattttagtacactgggcttgtaaaagcaagttatttatatatatcctataaatttaatttggatactgtatgttttgtctttactcttgcatgtgtataaaaaacataaaagtaagactattcaagct

SEQ ID NO: 54 - protein, 267 aa, Arabidopsis thaliana
MERDFLGLSDKQYLSNNVKHEVNDDAVEERGLSTKAAREWGKSKVFATSSFMPSSDFQEAKAFPGAYQWGSVSAANVFRRCQFGGAFQNATPLLLGGSVPLPTHPSLVPRVASSGSSPQLTIFYGGTISVFNDISPDKAQAIMLCAGNGLKGETGDSKPVREAERMYGKQIHNTAATSSSSATHTDNFSRCRDTPVAATNAMSMIESFNAAPRNMIPSVPQARKASLARFLEKRKERLMSAMPYKKMLLDLSTGESSGMNYSSTSPT

SEQ ID NO: 55 - DNA, 2297 bp, Arabidopsis thaliana
gcaaagagttaaataagcctctccaaaagtgtgtctgtaacattaccaaaacgaaaccttccttgtggattcccacttctttcttctgttttcttcttcctcttctttaaattggatgttttgggcaagaaacagagagaaacacgttaatttgagagtttgtcattgaatatttggtttgcaatggaaagagattttctgggtttgagcgacaagcagtatctaagtaataacgttaagcatgaggttaacgatgatgctgtcgaagaacgaggtttgtgttcttgtctcgagaatcttttattttaatgtttcaagaagagatcagttttcacttttaacatagccgtataaagttgtttatttaaatataatttttcagattccaaaacttgaaaaaaaaaagattccattaaatcttttataaaaatgagattggatagattagtcaaattgacgaccataaaaaatgatacttatagggttaagtacgaaggcagctagagaatgggggaagtcaaaggtttttgctacttcaagtttcatgccttcttcagatttccaggttggttcatcttaaaatttaacttactctgtatcagtttcagatgttatggctaatctaatggttctataagctaccgcataatcatggtcgtcttttagcatgtgcaagaggagtactcaattatggtcttgattaaaaagaagaatttactttcaaattatgttaaacacatcaatcacatatttatgagaaaagttgttttcgtaagagatagccaccggaaaatggtcggataaatggccgaactttatcatttttgtgtatgtggccaatcattaaccagggaaaaaaaattgttggataagtgctagttaagagctggtagggtcggtcgtctgccagccgcaaagttagggaaaaaataatttaatattttgtggcgtttggtgtttggcgtttggatcacgtttatttcttggcatttttctaaatttagaatgtacaaaaaatttaaagacgttgacgattaaaatttgaatttaacaaattaggaggctaaggcgtttccgggtgcataccagtggggatcagtttctgcggccaatgttttccgcagatgccaatttggtggtgcgtttcaaaacgcgacgccgcttttactaggcggttcagttcctttaccaactcatccttctcttgttccacggtaatttccatattatgatgcaaaaacattcaacaatttttttgctcttttcatattttgatttggttatgtgggtttgtggaaacagagtggcttcctccggatcatctcctcagctcacaatcttttatggcggaactataagcgtctttaatgacatatctcccgataaggtatatataatcaagattcatacaaataacatttacataacatttacatgttctaaaacggactattcatgatatgtgagtaggctcaagccatcatgttatgcgccgggaacggtttgaaaggtgaaactggagatagcaaaccggttcgagaagctgaaagaatgtatggaaaacaaatccataacactgctgctacctcatcaagctctgccactcacactgataatttctcaaggtgtagggacacacccgttgctgcgactaatgcaatgagcatgatcgaatcattcaatgcagctcctcgtaacatgattccttcaggtatgtgtgtctaatatcaacatcaaaacaaaatataatcaagatttttgcttcctcaaatcatatgtctaaactcgaaaattgcttttttccagtccctcaagctcggaaagcatccttggctcggttcttggagaagcgcaaagagaggtttgattttgtattttttttctttatagaaaattttgaggtttttcaattgaatctaaaagaattgatgttgttggtgcaggcttatgagtgcaatgccatacaagaagatgcttcttgatttgtcgaccggagaatccagtggaatgaattactcttctacttctcctacataaaacctacactttttttttttttttttacaatggtaatttgtaattgtaatcattagattatgattatatagttaccatttatattcttacgagcaggagaagacgttagggcgtctctgtatttgatcattgtttgtaatgctttggtctgtttattgtaggattacattataactttaagaactaacagatatatgtttgtcatggactcatgtctgtcaagaatttaatatcaaataaaattcactataatttttttt

SEQ ID NO: 56 - protein, 197 aa, Arabidopsis thaliana
MSKATIELDFLGLEKKQTNNAPKPKFQKFLDRRRSFRDIQGAISKIDPEIIKSLLASTGNNSDSSAKSRSVPSTPREDQPQIPISPVHASLARSSTELVSGTVPMTIFYNGSVSVFQVSRNKAGEIMKVANEAASKKDESSMETDLSVILPTTLRPKLFGQNLEGDLPIARRKSLQRFLEKRKERLVSTSPYYPTSA

SEQ ID NO: 57 - DNA, 1927 bp, Arabidopsis thaliana
aaaaactctcacatgagaaatcagaatccgttattattcctccatttattcatctcaaaacccatatctctctgtcttgatctctctctcactttctaataagatcaaagaagatgtcgaaagctaccatagaactcgatttcctcggacttgagaagaaacaaaccaacaacgctcctaagcctaagttccagaaatttctcgatcgccgtcgtagtttccgaggttcgtttggtttttagtcgctctctcttttttttttcttgcgataaatcgaatttattcatatggaactcctgcagatattcaaggtgcgatttcgaaaatcgatccggagattatcaaatcgctgttagcttccactggaaacaattccgattcatcggctaaatctcgttcggttccgtctactccgagggaagatcagcctcagatcccgatttctccggtccacgcgtctctcgccaggtatttttgtctttccggtaaagttttttttttctttctaacttttttggcgctaccagaaaagacgaaaaaatttgaaattcaaattttcaaaacattcattttcctcaggtctagtaccgaactcgtttcgggaactgttcctatgacgattttctacaatggaagtgtttcagttttccaagtgtctcgtaacaaagctggtgaaattatgaaggtcgctaatgaagcagcatctaagaaagacgagtcgtcgatggagacagatctttcggtaattcttccgaccactctaagaccaaagctctttggccagaatctagaaggaggttagtataataaaaataaaaatcacttagtgctggattcttctagaattttagttacatattattgcatgtagagatctaagaagagtttgttgttagagaggaattggttgctaattagtttggaattagatatcaaagagttaaagactatagtttatgtctatacgtattaatatacgttattaataaaagtataaacatgttgtttaatttctgataagaaactggtttatgcgtgtgtatgcagatcttcccatcgcaaggagaaagtcactgcaacgttttctcgagaagcgcaaggagaggtaatgattcttcaacaatccaaggatttttacccccaaataattaaagaaaggtttttatttttctctctctcgaccttttttttactataagttatttaagatagtaattatgggtcctgcctcttttactctcacatacaacttaagattcaactagttttgttcaacaacgcacatgcttatacgtagatagataatggagatcagtagtaatatcggtatacgtaggttactattgtaatggaacttttaaaaagcgcgttgactttgagtctttgactctagttctgtttgctacaccgacaagttatatttttcaaaatgatgagaaaacgaggagaaacaccggaaaaaaatttgaacttttacttttatcagaccatacggccaaagaaagatctgtatattatataagttatcacaaaacgcggtttcacattttctttttcgtcttgttgtgtttgcagattagtatcaacatctccttactatccgacatcggcctaaacgatctctttttagattgggacatggaccaaatttgtctttttcaatcggaagacatccatgttcgtttttggatttggcttatttccaatcttcttttgaagccttcttcgtcgttgctaaatcgtatactattcacgacaaacgtttttaggagattacgttacctactaagattatatatattggtttgtttttaaaaatgtctattatctttattgtcattgatagcttgatttaagaagctctctcttatcccgtgaccttctacttttgttttattttttagtatatggtaaagaaaattataac

SEQ ID NO: 58 - protein, 273 aa, Brassica rapa
MSSPMESSDFAATRRFSRKPSFSQTCSRLSQYLKENGSFGDLSLGMACKPEVNGISRQPTTTMSLFPCEASNMEPIGQDVKPKNLFPRQPSFSSSSSSLPKEDILKMTQATSSTRSVKPEPQTAPLTIFYGGQVIVFNDFSAEKAKEVMDLASKGTANTFTGFTSNVNNNIQSVYTTNLANNQTEMRSNIAPIPNQLPHLMKTTTQNPVQSSSTAMACELPIARRASLHRFLAKRKDRVTSKAPYQLNDPAKASSKPQTGDNTTSWLGLAAEM

SEQ ID NO: 59 - protein, 252 aa, Brassica oleracea
MSSSMECSTTRRSSSGKPSFSLTCSRLSQYLKENGSFGDLSLGMSCKPDTNGMSRKPTTTMSLFPCEASNVGSMAAAQDVKPKNLFPRQPSFSSSSSSIPKEDVPKMTQTTTRSLKPEPQTAPLTIFYGGQVIVFNDFSAEKAKEVMNLANKGTANTFTGFTSTLNNNIAPTPNQVPHLMKAATQDPKQTSSAAMACELPIARRASLHRFLAKRKDRVTSKAPYQLNDPAKAYSKPQTGNTTTSWLGLAADM

SEQ ID NO: 60 - protein, 233 aa, Zea mays
MAASARPGERATSFAVACSLLSRFVRQNGVAAADLGLRIKGEVEQQRTPATTNSLPGAEGEEVERRKETMELFPQSVGFSIKDAAAPREEQGDKEKPKQLTIFYGGKVLVFDDFPADKAKDLMQLASKGSPVVQNVALPQPSAAAAVTTDKAVLDPVISLAAAKKPARTNASDMPIMRKASLHRFLEKRKDRLNAKTPYQTAPSDAAPVKKEPESQPWLGLGPNAVDSSLNLS

SEQ ID NO: 61 - protein, 240 aa, Glycine max
MSSSSEYLVFSSHHPANSPAEKSTFSQTCSLLSQYIKEKGTFGDLTLGMTCTAETNGSPETSCHSATTMELFPTIITQRNPTTVDFLSPQTAYPHHSEVPIMVKSSAFKSMEKEPKAAQLTIFYAGQVVVFDDFPAEKLEEITSLAGKGISQSQNTSAYAHTHNQQVNHPSFVPNISPQAPSRPLVCDLPIARKASLHRFLSKRKDRIAAKAPYQINNPNSASSKPAESMSWLGLGAQST

SEQ ID NO: 62 - protein, 244 aa, Oryza sativa
MAASARPVGVGGERATSFAMACSLLSRYVRQNGAAAAELGLGIRGEGEAPRAAPATMSLLPGEAERKKETMELFPQSAGFGQQDAITADSAADAREQEPEKRQLTIFYGGKVLVFNDFPADKAKGLMQLASKGSPVAPQNAAAPAPAAVTDNTKAPMAVPAPVSSLPTAQADAQKPARANASDMPIARKASLHRFLEKRKDRLNAKTPYQASPSDATPVKKEPESQPWLGLGPNAVVKPIERGQ

SEQ ID NO: 63 - protein, 391 aa, Zea mays
MERDFLAAIGKEQQHPRKEKAGGGAEESAYFGAAAVPAMDWSFASKPCAAPALMSFRSAAREEPSFPQFSALDGTKNTAPRMLTHQRSFGPDSTQYAALHRAQNGARVVPVSSPFSQSNPMFRVQSSPSLPNSTAFKQPPFAISNAVASSTVGSYGGTRDAVRPRTAQLTIFYAGSVNVFNNVSAEKAQELMFLASRGSSAPVACKPEAPPTLAPAKVTAPEVLLPAKQMLFQKPQHLSPPPSSVPGILQSAALPRSASSSSNLDSPAPKSSVPLAVPPVSQAPPATLIATTTAAAIMPRAVPQARKASLARFLEKRKERVTTAAPYPSAKSPLESSDTFGSGSASANANDKSSCTDIALSSNHEESLCLGGQPRSIISFSEESPSTKLQI

SEQ ID NO: 64 - protein, 386 aa, Glycine max
MEREFFGLSSKNGAWTTMKDDAVNKSRDQVRSSGMQWSFPNKVSALPQFLSFKTNQEDKPRKTILEPLASSGYMAMSTQYAFDSNQKSFLGLTNRNLSISKHAAGNKQGMTVYPLQCCDAQSEEARIFSVSNQSNQVSPVLQSNLASTGLNMVNSVIKPQPFGSKSSGTPLSILPSIGSIVGSTDLRNNSKSSTMPTQLTIFYAGSVCVYDDISPEKAKAIMLMAGNGYTPTEKMELPTVKLQPAISIPSKDDGFMISQSYPPSTFPTPLPLTSHVNSQPGGGSSSNKEISIIRQVGPSTAPTNHLESPIIGSIGSASKEKAQPVCLPQARKASLARFLEKRKGRMMRTSPYLYMSKKSPECSSSGSDSVSFSLNFSGSCSLPATN

SEQ ID NO: 65 - protein, 416 aa, Oryza sativa
MERDFLGAIGKDEEQRRHAEERKESDYFGAGGGAAAAAMDWSFASRAALMSFRSSSSAAAAAAREETRELAFPHFSALDGAKMQQASHVLARQKSFGAESHGIPQYAAAAAVHGAHRGQPPHVLNGARVIPASSPFNPNNPMFRVQSSPNLPNAVGAGGGAFKQPPFAMGNAVAGSTVGVYGTRDMPKAKAAQLTIFYAGSVNVFNNVSPEKAQELMFLASRGSLPSAPTTVARMPEAHVFPPAKVTVPEVSPTKPMMLQKPQLVSSPVPAISKPISVVSQATSLPRSASSSNVDSNVTKSSGPLVVPPTSLPPPAQPETLATTTAAAIMPRAVPQARKASLARFLEKRKERVTTVAPYPLAKSPLESSDTMGSANDNKSSCTDIALSSNRDESLSLGQPRTISFCEESPSTKLQI

SEQ ID NO: 66 - protein, 404 aa, Zea mays
MAKSGASFPESSWMERDFLAAIGKEQQHPHKEEAGAEESAYFGGAGAAAAAPAMDWSFASKPGAAPALMSFRSASFPQFSSFDGAKNPAPRILTHQRSFGPDSTHYAAAHRTQHALNGARVTPVSSPFNQNSPMFRVQSSPSLPNGTAFKQPPFAINNNAAASSTVGFYGTRDVVRPKTAQLTIFYAGSVNVFDNVSAEKAQELMLLASRGSLPSSAPVARKPEAPILAPAKVTAPEVLHATQMLFQKPQHVSPPSSAISKPIPGILQAASLPRSASSSNLDSPFPKSSVPFPVSPVSQAPRAQPATIAATTAAAIMPRAVPQARKASLARFLEKRKERVTTAAPYPSAKSPMESSDTFGSGSANDKSSCTDIALSSNHEESLCLGQPRNISFIQESPSTKLQI

SEQ ID NO: 67 - protein, 340 aa, Glycine max
MERDFMGLNLKEPLAVVKEEMNNDGCKNSGFKKGRIAQWPFSNKVSALPHLMSFKASQDDKTKNTVSDTLSSSGFMSILSQEAFDTSQKRSAGEPQMFSVPNQAISVSLGNPFLKNHFAAAGQKPLLGGIPVTTSHSVLPSAVAVAGMTESCNSVKPSAQLTIFYAGTVNIFDDISAEKAQAIMLLAGNSLSAASNMAQPNVQVPISKLGAGAGVPVSQPANTSPGSGLSSPLSVSSHTGVQSGSGLTSTDEFLAAKTTGVPNTPICNVEPPKVVSATTMLTSAVPQARKASLARFLEKRKERVMSAAPYNLNKKSEECATAEYAGVNFSATNTVLAKQG

SEQ ID NO: 68 - protein, 427 aa, Oryza sativa
MERDFLGAIWRKEEAAGKPEEHSDYRGGGGGASAAMQWQFPATKVGAASSAFMSFRSSAAAAREEDPKEAAVFDRFSLSGFRPPPRPSPGDAFDGAAAMKQRQFGFNGRQQYAAAAQHGHREQGVDSYGVAAPHHFPSPSPSPRHPVPFGHANPMLRVHSLPNVAGGSPYRNQSFSVGNSVAGSTVGVYGGPRDLQNPKVTQMTIFYDGLVNVFDNIPVEKAQELMLLASRASIPSPPSAARKSDSPISAAAKLTVPEALPARQIVVQKPEASVPLVSGVSNPITIVSQAVTLPKSFSSSNDSAGPKSGGLPLAVTPLSQASPSQPIPVATTNASAIMPRAVPQARKASLARFLEKRKERVSSVAPYPSSKSPLESSDTIGSPSTPSKSSCTDITPSTNNCEDSLCLGQPRNISFSSQEPPSTKLQI

SEQ ID NO: 69 - protein, 353 aa, Zea mays
MDWSFASKPCAAPALMSFRSAAREEPSFPQFSALDGTKNTAPRMLTHQRSFGPDSTQYAALHRAQNGARVVPVSSPFSQSNPMFRVQSSPSLPNSTAFKQPPFAISNAVASSTVGSYGGTRDAVRPRTAQLTIFYAGSVNVFNNVSAEKAQELMFLASRGSSAPVACKPEAPPTLAPAKVTAPEVLLPAKQMLFQKPQHLSPPPSSVPGILQSAALPRSASSSSNLDSPAPKSSVPLAVPPVSQAPPATLIATTTAAAIMPRAVPQARKASLARFLEKRKERVTTAAPYPSAKSPLESSDTFGSGSASANANDKSSCTDIALSSNHEESLCLGGQPRSIISFSEESPSTKLQI

SEQ ID NO: 70 - protein, 338 aa, Glycine max
MERDFMGLNLKEPLAVVKEEMNNDGCKNSGFKKGRIAQWPFSNKVSALPHLMSFKASQDDKTKNTVSDTLSSSGFMSILSQEAFDTSQKRSAGEPQMFSVPNQAISVSLGNPFLKNHFAAAGQKPLLGGIPVTTSHSVLPSAVAVAGMTESCVKPSAQLTIFYAGTVNIFDDISAEKAQAIMLLAGNSLSAASNMAQPNVQVPISKLGAGAGVPVSQPANTSPGSGLSSPLSVSSHTGVQSGSGLTSTDEFLAAKTTGVPNTPICNVEPPKVVSATTMLTSAVPQARKASLARFLEKRKERVMSAAPYNLNKKSEECATAEYAGVNFSATNTVLAKQG

SEQ ID NO: 71 - protein, 308 aa, Oryza sativa
MQQASHVLARQPPHVLNGARVIPASSPFNPNNPMFRVQSSPNLPNAVGAGGGAFKQPPFAMGNAVAGSTVGVYGTRDMPKAKAAQLTIFYAGSVNVFNNVSPEKAQELMFLASRGSLPSAPTTVARMPEAHVFPPAKVTVPEVSPTKPMMLQKPQLVSSPVPAISKPISVVSQATSLPRSASSSNVDSNVTKSSGPLVVPPTSLPPPAQPETLATTTAAAIMPRAVPQARKASLARFLEKRKERVTTVAPYPLAKSPLESSDTMGSANDNKSSCTDIALSSNRDESLSLGQPRTISFCEESPSTKLQI

SEQ ID NO: 72 - protein, 218 aa, Zea mays
MAGHAPARDKTTTGFAATCSLLSQFLKEKKGGLQGLGGLAMAPAPAAGAGAFRPPTTMNLLSALDAAKATVGEPEGHGQRTGGNPREAAGEEAQQLTIFYGGKVVVFDRFPSAKVKDLLQIVSPPGADAVVDGAGAGAAVPTQNLPRPSHDSLSADLPIARRNSLHRFLEKRKDRITAKAPYQVNSSVGAEASKAEKPWLGLGQEQEGSDGRQAGEEM

SEQ ID NO: 73 - protein, 201 aa, Glycine max
MAAGVTVKSEVLESSPPEGVCSNTVENHLVQTNLSDGSPNKSVPASGLDAVIPSANQLTIFYNGSVCVYDGIPAEKVHEIMLIAAAAAKSTEMKKIGTQTTLISPAPSRPSSPHGITNNIGSSQKSSICRLQAEFPIARRHSLQRFLEKRRDRLGSKTPYPSSPTTKVADNIENNFCADNAPELISLNRSEEEFQPTVSAS

SEQ ID NO: 74 - protein, 188 aa, Oryza sativa
MSTRAPVELDFLGLRAAAADADDRHAKSGGSSASSSSSIRGMETSAIARIGPHLLRRVIAAAGPPPPPSTAPVPEEMPGAAAAAAPMTLFYNGSVAVFDVSHDKAEAIMRMATEATKAKGLARGNAIVGNFAKEPLTRTKSLQRFLSKRKERLTSLGPYQVGGPAAVGATTSTTTKSFLAKEEEHTAS

SEQ ID NO: 75 - DNA, 20 bp, Artificial Sequence
  A synthetic primer
accgagacacattcccgatt

SEQ ID NO: 76 - DNA, 20 bp, Artificial Sequence
  A synthetic primer
catcaggcttgcatgccatt

SEQ ID NO: 77 - DNA, 25 bp, Artificial Sequence
  A synthetic primer
acgaataagagcgtccattttagag

SEQ ID NO: 78 - DNA, 24 bp, Artificial Sequence
  A synthetic primer
gtggagtggtctaaagcaaccttc

SEQ ID NO: 79 - DNA, 23 bp, Artificial Sequence
  A synthetic primer
ataacgctgcggacatctacatt

SEQ ID NO: 80 - DNA, 21 bp, Artificial Sequence
  A synthetic primer
tcaggaagacagagtgttccc

SEQ ID NO: 81 - DNA, 21 bp, Artificial Sequence
  A synthetic primer
tgcgtttctctaagaaccgag

SEQ ID NO: 82 - skipped
  A synthetic primer

SEQ ID NO: 83 - DNA, 20 bp, Artificial Sequence
  A synthetic primer
ttgggtgatggttcacgtag

SEQ ID NO: 84 - DNA, 21 bp, Artificial Sequence
  A synthetic primer
taccgcataatcatggtcgtc

SEQ ID NO: 85 - DNA, 21 bp, Artificial Sequence
  A synthetic primer
tcatgctcattgcattagtcg

SEQ ID NO: 86 - DNA, 22 bp, Artificial Sequence
  A synthetic primer
ctttgaagacgtggttggaacg

SEQ ID NO: 87 - DNA, 22 bp, Artificial Sequence
  A synthetic primer
atttctcgatcgccgtcgtagt

SEQ ID NO: 88 - DNA, 25 bp, Artificial Sequence
  A synthetic primer
gccaaagagctttggtcttagagtg

SEQ ID NO: 89 - DNA, 25 bp, Artificial Sequence
  A synthetic primer
gtctaagcgtcaatttgtttacacc

SEQ ID NO: 90 - DNA, 25 bp, Artificial Sequence
  A synthetic primer
atgtcgagttctatggaatgttctg

SEQ ID NO: 91 - DNA, 26 bp, Artificial Sequence
  A synthetic primer
tcatatttcagctgctaaaccgagcc

SEQ ID NO: 92 - DNA, 21 bp, Artificial Sequence
  A synthetic primer
atggagagagattttctcggg

SEQ ID NO: 93 - DNA, 23 bp, Artificial Sequence
  A synthetic primer
ttaggttgcagagctgagagaag

SEQ ID NO: 94 - DNA, 20 bp, Artificial Sequence
  A synthetic primer
atggagagagattttctcgg

SEQ ID NO: 95 - DNA, 20 bp, Artificial Sequence
  A synthetic primer
cagatgatgagctggaggac

SEQ ID NO: 96 - DNA, 24 bp, Artificial Sequence
  A synthetic primer
atggaaagagattttctgggtttg

SEQ ID NO: 97 - DNA, 29 bp, Artificial Sequence
  A synthetic primer
ttatgtaggagaagtagaagagtaattca

SEQ ID NO: 98 - DNA, 22 bp, Artificial Sequence
  A synthetic primer
atgtcgaaagctaccatagaac

SEQ ID NO: 99 - DNA, 30 bp, Artificial Sequence
  A synthetic primer
gatagtaaggagatgttgatactaatctct

SEQ ID NO: 100 - DNA, 24 bp, Artificial Sequence
  A synthetic primer
atggctgatggtgaagacattcaa

SEQ ID NO: 101 - DNA, 24 bp, Artificial Sequence
  A synthetic primer
tcagaagcacttcctgtgaacaat

SEQ ID NO: 102 - DNA, 19 bp, Artificial Sequence
  A synthetic primer
aagcagcgtaatcggtagg

SEQ ID NO: 103 - DNA, 21 bp, Artificial Sequence
  A synthetic primer
gcacagcaatcgggtataaag

SEQ ID NO: 104 - DNA, 24 bp, Artificial Sequence
  A synthetic primer
ggagaactcacgatgggagcgatt

SEQ ID NO: 105 - DNA, 24 bp, Artificial Sequence
  A synthetic primer
gcgtcgtggctttcgataaccaga

SEQ ID NO: 106 - DNA, 17 bp, Artificial Sequence
  A synthetic primer
gctggcggttcgacatg

SEQ ID NO: 107 - DNA, 21 bp, Artificial Sequence
  A synthetic primer
gccattcctctgcgaattaga

SEQ ID NO: 108 - DNA, 26 bp, Artificial Sequence
  A synthetic primer
agaaactccaaatcaagaaccagctc

SEQ ID NO: 109 - DNA, 26 bp, Artificial Sequence
  A synthetic primer
ccggtttaatcgaagaacacgaagac

SEQ ID NO: 110 - protein, 4 aa, Artificial Sequence
  A synthetic protein
GWGD

SEQ ID NO: 111 - protein, 4 aa, Artificial Sequence
  A synthetic protein
DFSG

SEQ ID NO: 112 - protein, 11 aa, Artificial Sequence
  A synthetic protein
RELNSLISGGV

SEQ ID NO: 113 - protein, 10 aa, Artificial Sequence
  A synthetic protein
DTEWFFLVSM

SEQ ID NO: 114 - protein, 15 aa, Artificial Sequence
  A synthetic protein
VVNDLMIQQATVKMG

SEQ ID NO: 115 - protein, 32 aa, Artificial Sequence
  A synthetic protein
KRGRKPANGREEPLNHVEAERQRREKLNQRFY

SEQ ID NO: 116 - protein, 49 aa, Artificial Sequence
  A synthetic protein
GDNTVILGWGDGYYKGEEDKEKKKNNTNTAEQEHRKRVIRELNSLISGG

SEQ ID NO: 117 - protein, 51 aa, Artificial Sequence
  A synthetic protein
NNNTVLLGWGDGYYKGEEEKSRKKKSNPASAAEQEHRKRVIRELNSLISGG

SEQ ID NO: 118 - protein, 52 aa, Artificial Sequence
  A synthetic protein
GAGASLLGWGDGYYKGCDDADKRARQQPTPASAAEQHRKRVLRELNSLIAGG

SEQ ID NO: 119 - protein, 53 aa, Artificial Sequence; identical to SEQ ID NO: 12
  A synthetic protein

SEQ ID NO: 120 - protein, 53 aa, Artificial Sequence
  A synthetic protein
STGASLLGWGDGYYKGCDDDKRKQRSSTPAAAAEQEHRKRVLRRELNSLIAGA

SEQ ID NO: 121 - protein, 52 aa, Artificial Sequence; identical to SEQ ID NO: 10
  A synthetic protein

SEQ ID NO: 122 - protein, 52 aa, Artificial Sequence
  A synthetic protein
ATGASLLGWGDGYYKGCDDDKRKQRPLTPAAQAEQEHRKRVLRELNSLISGA

SEQ ID NO: 123 - protein, 55 aa, Artificial Sequence
  A synthetic protein
FSGASVLGWGDHYYKGEEDKAKPRQRSSSPPFSTPADQEYRKKVLRELNSLISGG

SEQ ID NO: 124 - protein, 55 aa, Artificial Sequence
  A synthetic protein
FSGASVLGWGDGYYKGEEDKANPRRRSSSPPFSTPADQEYRKKVLRELNSLISGG

SEQ ID NO: 125 - protein, 53 aa, Artificial Sequence; identical to SEQ ID NO: 20
  A synthetic protein

SEQ ID NO: 126 - protein, 54 aa, Artificial Sequence
  A synthetic protein
FASQTVLGWGDGYYKGEEDKNKRRGSSSSAANFCAEQEHRKKVLRELNSLISGV

SEQ ID NO: 127 - protein, 55 aa, Artificial Sequence
  A synthetic protein
RSGQQVLGWGDGCCREPNEEEESKVVRSYNFNNMGAEEETWQDMRKRVLQKLHRL

SEQ ID NO: 128 - protein, 55 aa, Artificial Sequence
  A synthetic protein
KAGDLVLCWGDGYCREPKEGEKSEIVRILSMGREEETHQTMRKRVLQKLHDLFGG